European Patent Specification EP 2 968 546 B1, published September 20, 2023. Title: Methods of Generating Bioactive Peptide-bearing Antibodies and Compositions Comprising the Same. Applicant: Omeros Corporation Cummings, W. Jason Gray, Pat Tjoelker, Larry Yabuki, Munehisa. The sequence listing filed with the application follows.

SEQUENCE LISTING (195 sequences)

SEQ ID NO: 1 - DNA, 6476 bp, Homo Sapiens
acacacagagtgatacaaatacctgcttgagcccctcagttattttctctcaagggctgaagtcagccacacaggataaaggagggaagggaaggagcagatcttttcggtaggaagacagattttgttgtcaggttcctgggagtgcaagagcaagtcaaaggagagagagaggagagaggaaaagccagagggagagagggggagaggggatctgttgcaggcaggggaaggcgtgacctgaatggagaatgccagccaattccagagacacacagggacctcagaacaaagataaggcatcacggacaccacaccgggcacgagctcacaggcaagtcaagctgggaggaccaaggccgggcagccgggagcacccaaggcaggaaaatgaggtggctgcttctctattatgctctgtgcttctccctgtcaaaggcttcagcccacaccgtggagctaaacaatatgtttggccagatccagtcgcctggttatccagactcctatcccagtgattcagaggtgacttggaatatcactgtcccagatgggtttcggatcaagctttacttcatgcacttcaacttggaatcctcctacctttgtgaatatgactatgtgaaggtagaaactgaggaccaggtgctggcaaccttctgtggcagggagaccacagacacagagcagactcccggccaggaggtggtcctctcccctggctccttcatgtccatcactttccggtcagatttctccaatgaggagcgtttcacaggctttgatgcccactacatggctgtggatgtggacgagtgcaaggagagggaggacgaggagctgtcctgtgaccactactgccacaactacattggcggctactactgctcctgccgcttcggctacatcctccacacagacaacaggacctgccgagtggagtgcagtgacaacctcttcactcaaaggactggggtgatcaccagccctgacttcccaaacccttaccccaagagctctgaatgcctgtataccatcgagctggaggagggtttcatggtcaacctgcagtttgaggacatatttgacattgaggaccatcctgaggtgccctgcccctatgactacatcaagatcaaagttggtccaaaagttttggggcctttctgtggagagaaagccccagaacccatcagcacccagagccacagtgtcctgatcctgttccatagtgacaactcgggagagaaccggggctggaggctctcatacagggctgcaggaaatgagtgcccagagctacagcctcctgtccatgggaaaatcgagccctcccaagccaagtatttcttcaaagaccaagtgctcgtcagctgtgacacaggctacaaagtgctgaaggataatgtggagatggacacattccagattgagtgtctgaaggatgggacgtggagtaacaagattcccacctgtaaaattgtagactgtagagccccaggagagctggaacacgggctgatcaccttctctacaaggaacaacctcaccacatacaagtctgagatcaaatactcctgtcaggagccctattacaagatgctcaacaataacacaggtatatatacctgttctgcccaaggagtctggatgaataaagtattggggagaagcctacccacctgccttccagtgtgtgggctccccaagttctcccggaagctgatggccaggatcttcaatggacgcccagcccagaaaggcaccactccctggattgccatgctgtcacacctgaatgggcagcccttctgcggaggctcccttctaggctccagctggatcgtgaccgccgcacactgcctccaccagtcactcgatccggaagatccgaccctacgtgattcagacttgctcagcccttctgacttcaaaatcatcctgggcaagcattggaggctccggtcagatgaaaatgaacagcatctcggcgtcaaacacaccactctccacccccagtatgatcccaacacattcgagaatgacgtggctctggtggagctgttggagagcccagtgctgaatgccttcgtgatgcccatctgtctgcctgagggaccccagcaggaaggagccatggtcatcgtcagcggctgggggaagcagttcttgcaaaggttcccagagaccctgatggagattgaaatcccgattgttgaccacagcacctgccagaaggcttatgccccgctgaagaagaaagtgaccagggacatgatctgtgctggggagaaggaagggggaaaggacgcctgtgcgggtgactctggaggccccatggtgaccctgaatagagaaagaggccagtggtacctggtgggcactgtgtcctggggtgatgactgtgggaagaaggaccgctacggagtatactcttacatccaccacaacaaggactggatccagagggtcaccggagtgaggaactgaatttggctcctcagccccagcaccaccagctgtgggcagtcagtagcagaggacgatcctccgatgaaagcagccatttctcctttccttcctcccatcccccctccttcggcctatccattactgggcaatagagcaggtatcttcacccccttttcactctctttaaagagatggagcaagagagtggtcagaacacaggccgaatccaggctctatcacttactagtttgcagtgctgggcaggtgacttcatctcttcgaacttcagtttcttcataagatggaaatgctataccttacctacctcgtaaaagtctgatgaggaaaagattaactaatagatgcatagcacttaacagagtgcatagcatacactgttttcaataaatgcaccttagcagaaggtcgatgtgtctaccaggcagacgaagctctcttacaaacccctgcctgggtcttagcattgatcagtgacacacctctcccctcaaccttgaccatctccatctgcccttaaatgctgtatgcttttttgccaccgtgcaacttgcccaacatcaatcttcaccctcatccctaaaaaagtaaaacagacaaggttctgagtcctgtggtatgtcccctagcaaatgtaactaggaacatgcactagatgacagattgcgggagggcctgagagaagcagggacaggagggagcctggggattgtggtttgggaaggcagacacctggttctagaactagctctgcccttagccccctgtatgaccctatgcaagtcctcctccctcatctcaaagggtcctcaaagctctgacgatctaagatacaatgaagccattttccccctgataagatgaggtaaagccaatgtaaccaaaaggcaaaaattacaatcggttcaaaggaactttgatgcagacaaaatgctgctgctgctgctcctgaaatacccacccctttccactacgggtgggttcccaaggacatgggacaggcaaagtgtgagccaaaggatccttccttattcctaagcagagcatctgctctgggccctggcctccttcccttcttgggaaactgggctgcatgaggtgggccctggtagtttgtaccccaggcccctatactcttccttcctatgtccacagctgaccccaagcagccgttccccgactcctcacccctgagcctcaccctgaactccctcatcttgcaaggccataagtgttttccaagcaaaatgcctctcccatcctctctcaggaagcttctagagactttatgccctccagagctccaagatataagccctccaagggatcagaagctccaagttcctgtcttctgttttatagaaattgatcttccctgggggactttaactcttgacctgtatgcagctgttggagtaattccaggtctcttgaaaaaaaagaggaagataatggagaatgagaacatatatatatatatattaagccccaggctgaatactcagggacagcaattcacagcctgcctctggttctataaacaagtcattctacctctttgtgccctgctgtttattctgtaaggggaaggtggcaatgggacccagctccatcagacacttgtcaagctagcagaaactccattttcaatgccaaagaagaactgtaatgctgttttggaatcatcccaaggcatcccaagacaccatatcttcccatttcaagcactgcctgggcacaccccaacatcccaggctgtggtggctcctgtgggaactacctagatgaagagagtatcatttataccttctaggagctcctattgggagacatgaaacatatgtaattgactaccatgtaatagaacaaaccctgccaagtgctgctttggaaagtcatggaggtaaaagaaagaccattctggtatgaaggttttgggggaggagatatcaatcaagaaggcttcccagaagaggtgactggaccagagccttgtccacaggtaagacggaggaggccttccacatggagggagaacaatagtaaatgtccactcaagatgtcctttattataccagctcctcccacaaaaacacatgtccagtggactctttttctgggatcagaaccaacaccaaaaagagcttttctccttaaagttagaattctaaacaggacttgaaatggcctcaaggtttgtgcacaaatactgacttctggctggacccagcttattctgtttatttctccaattgcaatttcatccttatcctgagaaaatgtctaaataggccatggaacccaggcttccccgtgacctacaagcacttattagctgtgccagctcctgcactgctgctaaggtccaagaaacccagatctctcacagagccatagaagcagagggctggagtatctgtgaggacaacaaccttgtctaacttcgcgacctcattcttgagcatttctactgatgagaaactcactacccccaattgcagctcattcaactttaaaattgctgctttttgaatcactgattgtgaatattaatttaaaaaaataagtaagaaaatgttttaaatgtgctgcctctttaaaaggtctcctctttgtgcaaccaaaacccacctctctagaatacagtttgtataactgaagctataatttcataccatgagtgctgctgttagcaataataatcatgcccggattttattaacaacagaagctgttgctcgtatgaaaaaacaaacattagttctaataaacatctgcattgagtcaaagctccctgtttgtttgtatgtcttttatgcactgatgattatagtgagttgctttcatttaccaacattttgttgtattcgtgtaggatcactgtaccatgaagggagagagactatgatgggaagattgttgtagatacaaaagcatgtcttaggtttttgggtcagttctgtttaaatacctgtcctattattcctgtaaattatcaaaatatcccagaatgtcaatgtttctgcatccacattacaattattaaatgccactcatttattaaatttactattatcagtggcatttaataaatttgaatcatatgttcagtgtttggtttagaaaatatggtgccatgtctatgagtggcctgttctggattggagtacatgccttctttctgccttgagttaatcttactcaatggagaacaagaatcaaagaaacaccaccaccaagaagcccttcaagctagagttgggcaagagtcagggaggggaatgtagaccactcatatgacagaggtggaaaccaatcttggtctagaataagtctcaaaatcaaaagacttgaattctagtgcagcgtaggttgactcccttatttatttaattttcccatctctacaccgctagaataacctctctcctgaggctgttgaatctgatgaattagcagataggaaagaacttagaaaattataagttcactcaaatgtaaaaggttatatgggaaataatcaccactaacatttttgagtacttactatctgcttgttatacacattctctaatttaattttcacaagaaaattcatgaaaggactatacttatcccccttttacaggtgagcaacctggagtgcagtgaagtgtaaaatgtgggccgacttaggagcacaaataccccagcaacaatgagcactcttagtacacaggtcttggtttctaaaatatcatcatccgataaaaggaacacaggctctttgaagaaatgactgattccgggattggggcaagaaacacacaagctgagactggagcatcttgcagtcccagaaagtgaagaaacgctgaggatatgtcaaagggacacaggagccaaatgaaagagcttccactggccaaagctggaatgttgagcaacaaagcaacatagcattggataataacccaaagtataaaataaatattcatgagtacata

SEQ ID NO: 2 - protein, 699 aa, Homo Sapiens
MRWLLLYYALCFSLSKASAHTVELNNMFGQIQSPGYPDSYPSDSEVTWNITVPDGFRIKLYFMHFNLESSYLCEYDYVKVETEDQVLATFCGRETTDTEQTPGQEVVLSPGSFMSITFRSDFSNEERFTGFDAHYMAVDVDECKEREDEELSCDHYCHNYIGGYYCSCRFGYILHTDNRTCRVECSDNLFTQRTGVITSPDFPNPYPKSSECLYTIELEEGFMVNLQFEDIFDIEDHPEVPCPYDYIKIKVGPKVLGPFCGEKAPEPISTQSHSVLILFHSDNSGENRGWRLSYRAAGNECPELQPPVHGKIEPSQAKYFFKDQVLVSCDTGYKVLKDNVEMDTFQIECLKDGTWSNKIPTCKIVDCRAPGELEHGLITFSTRNNLTTYKSEIKYSCQEPYYKMLNNNTGIYTCSAQGVWMNKVLGRSLPTCLPVCGLPKFSRKLMARIFNGRPAQKGTTPWIAMLSHLNGQPFCGGSLLGSSWIVTAAHCLHQSLDPEDPTLRDSDLLSPSDFKIILGKHWRLRSDENEQHLGVKHTTLHPQYDPNTFENDVALVELLESPVLNAFVMPICLPEGPQQEGAMVIVSGWGKQFLQRFPETLMEIEIPIVDHSTCQKAYAPLKKKVTRDMICAGEKEGGKDACAGDSGGPMVTLNRERGQWYLVGTVSWGDDCGKKDRYGVYSYIHHNKDWIQRVTGVRN

SEQ ID NO: 3 - DNA, 2471 bp, Homo Sapiens
agaccaggccaggccagctggacgggcacaccatgaggctgctgaccctcctgggccttctgtgtggctcggtggccacccccttgggcccgaagtggcctgaacctgtgttcgggcgcctggcatcccccggctttccaggggagtatgccaatgaccaggagcggcgctggaccctgactgcaccccccggctaccgcctgcgcctctacttcacccacttcgacctggagctctcccacctctgcgagtacgacttcgtcaagctgagctcgggggccaaggtgctggccacgctgtgcgggcaggagagcacagacacggagcgggcccctggcaaggacactttctactcgctgggctccagcctggacattaccttccgctccgactactccaacgagaagccgttcacggggttcgaggccttctatgcagccgaggacattgacgagtgccaggtggccccgggagaggcgcccacctgcgaccaccactgccacaaccacctgggcggtttctactgctcctgccgcgcaggctacgtcctgcaccgtaacaagcgcacctgctcagccctgtgctccggccaggtcttcacccagaggtctggggagctcagcagccctgaatacccacggccgtatcccaaactctccagttgcacttacagcatcagcctggaggaggggttcagtgtcattctggactttgtggagtccttcgatgtggagacacaccctgaaaccctgtgtccctacgactttctcaagattcaaacagacagagaagaacatggcccattctgtgggaagacattgccccacaggattgaaacaaaaagcaacacggtgaccatcacctttgtcacagatgaatcaggagaccacacaggctggaagatccactacacgagcacagcgcagccttgcccttatccgatggcgccacctaatggccacgtttcacctgtgcaagccaaatacatcctgaaagacagcttctccatcttttgcgagactggctatgagcttctgcaaggtcacttgcccctgaaatcctttactgcagtttgtcagaaagatggatcttgggaccggccaatgcccgcgtgcagcattgttgactgtggccctcctgatgatctacccagtggccgagtggagtacatcacaggtcctggagtgaccacctacaaagctgtgattcagtacagctgtgaagagaccttctacacaatgaaagtgaatgatggtaaatatgtgtgtgaggctgatggattctggacgagctccaaaggagaaaaatcactcccagtctgtgagcctgtttgtggactatcagcccgcacaacaggagggcgtatatatggagggcaaaaggcaaaacctggtgattttccttggcaagtcctgatattaggtggaaccacagcagcaggtgcacttttatatgacaactgggtcctaacagctgctcatgccgtctatgagcaaaaacatgatgcatccgccctggacattcgaatgggcaccctgaaaagactatcacctcattatacacaagcctggtctgaagctgtttttatacatgaaggttatactcatgatgctggctttgacaatgacatagcactgattaaattgaataacaaagttgtaatcaatagcaacatcacgcctatttgtctgccaagaaaagaagctgaatcctttatgaggacagatgacattggaactgcatctggatggggattaacccaaaggggttttcttgctagaaatctaatgtatgtcgacataccgattgttgaccatcaaaaatgtactgctgcatatgaaaagccaccctatccaaggggaagtgtaactgctaacatgctttgtgctggcttagaaagtgggggcaaggacagctgcagaggtgacagcggaggggcactggtgtttctagatagtgaaacagagaggtggtttgtgggaggaatagtgtcctggggttccatgaattgtggggaagcaggtcagtatggagtctacacaaaagttattaactatattccctggatcgagaacataattagtgatttttaacttgcgtgtctgcagtcaaggattcttcatttttagaaatgcctgtgaagaccttggcagcgacgtggctcgagaagcattcatcattactgtggacatggcagttgttgctccacccaaaaaaacagactccaggtgaggctgctgtcatttctccacttgccagtttaattccagccttacccattgactcaaggggacataaaccacgagagtgacagtcatctttgcccacccagtgtaatgtcactgctcaaattacatttcattaccttaaaaagccagtctcttttcatactggctgttggcatttctgtaaactgcctgtccatgctctttgtttttaaacttgttcttattgaaaaaaaaaaaaaaaaa

SEQ ID NO: 4 - protein, 686 aa, Homo Sapiens
MRLLTLLGLLCGSVATPLGPKWPEPVFGRLASPGFPGEYANDQERRWTLTAPPGYRLRLYFTHFDLELSHLCEYDFVKLSSGAKVLATLCGQESTDTERAPGKDTFYSLGSSLDITFRSDYSNEKPFTGFEAFYAAEDIDECQVAPGEAPTCDHHCHNHLGGFYCSCRAGYVLHRNKRTCSALCSGQVFTQRSGELSSPEYPRPYPKLSSCTYSISLEEGFSVILDFVESFDVETHPETLCPYDFLKIQTDREEHGPFCGKTLPHRIETKSNTVTITFVTDESGDHTGWKIHYTSTAQPCPYPMAPPNGHVSPVQAKYILKDSFSIFCETGYELLQGHLPLKSFTAVCQKDGSWDRPMPACSIVDCGPPDDLPSGRVEYITGPGVTTYKAVIQYSCEETFYTMKVNDGKYVCEADGFWTSSKGEKSLPVCEPVCGLSARTTGGRIYGGQKAKPGDFPWQVLILGGTTAAGALLYDNWVLTAAHAVYEQKHDASALDIRMGTLKRLSPHYTQAWSEAVFIHEGYTHDAGFDNDIALIKLNNKVVINSNITPICLPRKEAESFMRTDDIGTASGWGLTQRGFLARNLMYVDIPIVDHQKCTAAYEKPPYPRGSVTANMLCAGLESGGKDSCRGDSGGALVFLDSETERWFVGGIVSWGSMNCGEAGQYGVYTKVINYIPWIENIISDF

SEQ ID NO: 5 - protein, 9 aa, Artificial Sequence
  Synthetic
  VARIANT (1)..(1): wherein Xaa at position 1 is Phe or Val
  VARIANT (4)..(4): wherein Xaa at position 4 is Arg or Lys
  VARIANT (5)..(5): wherein Xaa at position 5 is Lys or Leu
  VARIANT (6)..(6): wherein Xaa at position 6 is Leu or Trp
  VARIANT (8)..(8): wherein Xaa at position 8 is Tyr or Asn
XCTXXXCXQ

SEQ ID NO: 6 - protein, 36 aa, Artificial Sequence
  Synthetic
LEVTCEPGTTFKDKCNTCRCGSDGKSAFCTRKLCYQ

SEQ ID NO: 7 - protein, 33 aa, Artificial Sequence
  Synthetic
TCEPGTTFKDKCNTCRCGSDGKSAFCTRKLCYQ

SEQ ID NO: 8 - protein, 20 aa, Artificial Sequence
  Synthetic
TCRCGSDGKSAFCTRKLCYQ

SEQ ID NO: 9 - protein, 36 aa, Artificial Sequence
  Synthetic
LEVTCEPGTTFKDKCNTCRCGSDGKSAVCTKLWCNQ

SEQ ID NO: 10 - protein, 33 aa, Artificial Sequence
  Synthetic
TCEPGTTFKDKCNTCRCGSDGKSAVCTKLWCNQ

SEQ ID NO: 11 - protein, 20 aa, Artificial Sequence
  Synthetic
TCRCGSDGKSAVCTKLWCNQ

SEQ ID NO: 12 - protein, 227 aa, Homo Sapiens
DKTHTCPPCPAPELLGGPSVFLFPPKPKDTLMISRTPEVTCVVVDVSHEDPEVKFNWYVDGVEVHNAKTKPREEQYNSTYRVVSVLTVLHQDWLNGKEYKCKVSNKALPAPIEKTISKAKGQPREPQVYTLPPSREEMTKNQVSLTCLVKGFYPSDIAVEWESNGQPENNYKTTPPVLDSDGSFFLYSKLTVDKSRWQQGNVFSCSVMHEALHNHYTQKSLSLSPGK

SEQ ID NO: 13 - protein, 12 aa, Artificial Sequence
  Synthetic
GTGGGSGSSSRS

SEQ ID NO: 14 - protein, 10 aa, Artificial Sequence
  Synthetic
GTGGGSGSSS

SEQ ID NO: 15 - DNA, 888 bp, Artificial Sequence
  Synthetic
atgtacaggatgcaactcctgtcttgcattgcactaagtcttgcacttgtcacgaattcgctcgaggtgacatgtgaacccggtacgacgtttaaggataagtgcaacacatgtaggtgcggtagcgacggcaaatcagcgttctgtacccggaaattgtgctaccagggaactggaggagggtcggggtcctcgtcaagatctgacaaaactcacacatgcccaccgtgcccagcacctgaactcctggggggaccgtcagtcttcctcttccccccaaaacccaaggacaccctcatgatctcccggacccctgaggtcacatgcgtggtggtggacgtgagccacgaagaccctgaggtcaagttcaactggtacgtggacggcgtggaggtgcataatgccaagacaaagccgcgggaggagcagtacaacagcacgtaccgtgtggtcagcgtcctcaccgtcctgcaccaggactggctgaatggcaaggagtacaagtgcaaggtctccaacaaagccctcccagcccccatcgagaaaaccatctccaaagccaaagggcagccccgagaaccacaggtgtacaccctgcccccatcccgggaggagatgaccaagaaccaggtcagcctgacctgcctggtcaaaggcttctatcccagcgacatcgccgtggagtgggagagcaatgggcagccggagaacaactacaagaccacgcctcccgtgctggactccgacggctccttcttcctctacagcaagctcaccgtggacaagagcaggtggcagcaggggaacgtcttctcatgctccgtgatgcacgaggctctgcacaaccactacacgcagaagagcctctccctgtctccgggtaaatga

SEQ ID NO: 16 - protein, 275 aa, Artificial Sequence
  Synthetic
LEVTCEPGTTFKDKCNTCRCGSDGKSAFCTRKLCYQGTGGGSGSSSRSDKTHTCPPCPAPELLGGPSVFLFPPKPKDTLMISRTPEVTCVVVDVSHEDPEVKFNWYVDGVEVHNAKTKPREEQYNSTYRVVSVLTVLHQDWLNGKEYKCKVSNKALPAPIEKTISKAKGQPREPQVYTLPPSREEMTKNQVSLTCLVKGFYPSDIAVEWESNGQPENNYKTTPPVLDSDGSFFLYSKLTVDKSRWQQGNVFSCSVMHEALHNHYTQKSLSLSPGK

SEQ ID NO: 17 - DNA, 888 bp, Artificial Sequence
  Synthetic
atgtacaggatgcaactcctgtcttgcattgcactaagtcttgcacttgtcacgaattcgttggaagtgacgtgtgagcccggaacgacattcaaagacaagtgcaatacttgtcggtgcggttcagatgggaaatcggcggtctgcacaaagctctggtgtaaccagggcaccggtggagggtcgggatccagctcaagatctgacaaaactcacacatgcccaccgtgcccagcacctgaactcctggggggaccgtcagtcttcctcttccccccaaaacccaaggacaccctcatgatctcccggacccctgaggtcacatgcgtggtggtggacgtgagccacgaagaccctgaggtcaagttcaactggtacgtggacggcgtggaggtgcataatgccaagacaaagccgcgggaggagcagtacaacagcacgtaccgtgtggtcagcgtcctcaccgtcctgcaccaggactggctgaatggcaaggagtacaagtgcaaggtctccaacaaagccctcccagcccccatcgagaaaaccatctccaaagccaaagggcagccccgagaaccacaggtgtacaccctgcccccatcccgggaggagatgaccaagaaccaggtcagcctgacctgcctggtcaaaggcttctatcccagcgacatcgccgtggagtgggagagcaatgggcagccggagaacaactacaagaccacgcctcccgtgctggactccgacggctccttcttcctctacagcaagctcaccgtggacaagagcaggtggcagcaggggaacgtcttctcatgctccgtgatgcacgaggctctgcacaaccactacacgcagaagagcctctccctgtctccgggtaaatga

SEQ ID NO: 18 - protein, 275 aa, Artificial Sequence
  Synthetic
LEVTCEPGTTFKDKCNTCRCGSDGKSAVCTKLWCNQGTGGGSGSSSRSDKTHTCPPCPAPELLGGPSVFLFPPKPKDTLMISRTPEVTCVVVDVSHEDPEVKFNWYVDGVEVHNAKTKPREEQYNSTYRVVSVLTVLHQDWLNGKEYKCKVSNKALPAPIEKTISKAKGQPREPQVYTLPPSREEMTKNQVSLTCLVKGFYPSDIAVEWESNGQPENNYKTTPPVLDSDGSFFLYSKLTVDKSRWQQGNVFSCSVMHEALHNHYTQKSLSLSPGK

SEQ ID NO: 19 - DNA, 30 bp, Artificial Sequence
  Synthetic
ctactgcgccaaactcgaggtgacatgtga

SEQ ID NO: 20 - DNA, 30 bp, Artificial Sequence
  Synthetic
cgtggccccatgcctggtagcacaatttcc

SEQ ID NO: 21 - DNA, 30 bp, Artificial Sequence
  Synthetic
cgggggtggcagcttggaagtgacgtgtga

SEQ ID NO: 22 - DNA, 30 bp, Artificial Sequence
  Synthetic
agccataatagtactggttacaccagagct

SEQ ID NO: 23 - protein, 125 aa, Chicken
AVTLDESGGGLQTPGRALSLVCKASGFTFSSYNMGWVRQAPGKGLEFVAGIDNTGRYTGYGSAVKGRATISRDNGQSTVRLQLNNLRAEDTGTYYCAKAAGGSGYCGSGAYIDAWGHGTEVIVSS

SEQ ID NO: 24 - protein, 30 aa, Chicken
  VARIANT (16)..(16): wherein Xaa at position 16 is Arg or Gly
AVTLDESGGGLQTPGXALSLVCKASGFTFS

SEQ ID NO: 25 - protein, 14 aa, Chicken
  VARIANT (12)..(12): wherein Xaa at position 12 is Phe or Trp
WVRQAPGKGLEXVA

SEQ ID NO: 26 - protein, 32 aa, Chicken
  VARIANT (13)..(13): wherein Xaa at position 13 is Val or Leu
  VARIANT (31)..(31): wherein Xaa at position 31 is Ala or Thr
RATISRDNGQSTXRLQLNNLRAEDTGIYYCXK

SEQ ID NO: 27 - protein, 5 aa, Chicken
  VARIANT (4)..(4): wherein Xaa at position 4 is Ala or Thr
YYCXK

SEQ ID NO: 28 - protein, 11 aa, Chicken
WGHGTEVIVSS

SEQ ID NO: 29 - protein, 5 aa, Chicken
WGHGT

SEQ ID NO: 30 - protein, 102 aa, Chicken
ALTQPSSVSANPGGTVKITCSGDSSYYGWYQQKAPGSAPVTVIYDNTNRPSNIPSRFSGSKSGSTATLTITGVRADDNAVYYCASTDSSSTAFGAGTTLTVL

SEQ ID NO: 31 - protein, 20 aa, Chicken
  VARIANT (6)..(6): wherein Xaa at position 6 is Ala or Ser
  VARIANT (12)..(12): wherein Xaa at position 12 is Leu or Pro
  VARIANT (14)..(14): wherein Xaa at position 14 is Gly or Glu
ALTQPXSVSANXGXTVKITC

SEQ ID NO: 32 - protein, 5 aa, Chicken
VKITC

SEQ ID NO: 33 - protein, 16 aa, Chicken
  VARIANT (6)..(6): wherein Xaa at position 6 is Ala or Ser
  VARIANT (14)..(14): wherein Xaa at position 14 is Val or Leu
WYQQKXPGSAPVTXIY

SEQ ID NO: 34 - protein, 5 aa, Chicken
  MISC_FEATURE (2)..(2): Wherein Xaa is Tyr or Phe or His
WXQQK

SEQ ID NO: 35 - protein, 32 aa, Chicken
  VARIANT (1)..(1): wherein Xaa at position 1 is Asn or Asp
  VARIANT (10)..(10): wherein Xaa at position 10 is Lys or Leu
  VARIANT (15)..(15): Wherein Xaa at position 15 is Ala or Asn
  VARIANT (27)..(27): wherein Xaa at position 27 is Asn or Glu
  VARIANT (31)..(31): Wherein Xaa at position 31 is Tyr or Phe
XIPSRFSGSXSGSTXTLTITGVRADDXAVYXC

SEQ ID NO: 36 - protein, 10 aa, Chicken
FGAGTTLTVL

SEQ ID NO: 37 - protein, 6 aa, Artificial Sequence
  Synthetic
AAGGSG

SEQ ID NO: 38 - protein, 10 aa, Artificial Sequence
  Synthetic
AAGGSGGSGA

SEQ ID NO: 39 - protein, 4 aa, Artificial Sequence
  Synthetic
YIDA

SEQ ID NO: 40 - protein, 5 aa, Artificial Sequence
  Synthetic
AYIDA

SEQ ID NO: 41 - protein, 14 aa, Artificial Sequence
  Synthetic
GTGGGSGSSSYIDA

SEQ ID NO: 42 - protein, 8 aa, Artificial Sequence
  Synthetic
GSGAYIDA

SEQ ID NO: 43 - protein, 14 aa, Artificial Sequence
  Synthetic
AAGGSGGSGAYIDA

SEQ ID NO: 44 - protein, 5 aa, Artificial Sequence
  Synthetic
SGGGS

SEQ ID NO: 45 - protein, 4 aa, Artificial Sequence
  Synthetic
YYYG

SEQ ID NO: 46 - protein, 4 aa, Artificial Sequence
  Synthetic
GSGA

SEQ ID NO: 47 - protein, 330 aa, Homo Sapiens [sequence omitted]

SEQ ID NO: 48 - DNA, 1488 bp, Artificial Sequence
  Synthetic
atggagttcggcctgagctggctgttcctggtggccatccttaagggcgtgcagtgcgccgtgacgttggacgagtccgggggcggcctccagacgcccgggggagcgctcagcctcgtctgcaaggcctccgggttcaccttcagcagtaacgccatgggttgggtgcgacaggcgcccggcaaggggctggagtgggtcgctggtattgatgatgatggtagtggcacaagatacgcgccggcggtgaagggccgtgccaccatctcgagggacaacgggcagagcacactgaggctgcagctgaacaacctcagggctgaggacaccggcacctactactgcgccaaactcgaggtgacatgtgaacccggtacgacgtttaaggataagtgcaacacatgtaggtgcggtagcgacggcaaatcagcgttctgtacccggaaattgtgctaccaggcatggggccacgggaccgaagtcatcgtctcctccgctagcaccaagggcccatcggtcttccccctggcaccctcctccaagagcacctctgggggcacagcggccctgggctgcctggtcaaggactacttccccgaaccggtgacggtgtcgtggaactcaggcgccctgaccagcggcgtgcacaccttcccggctgtcctacagtcctcaggactctactccctcagcagcgtggtgaccgtgccctccagcagcttgggcacccagacctacatctgcaacgtgaatcacaagcccagcaacaccaaggtggacaagaaagttgagcccaaatcttgtgacaaaactcacacatgcccaccgtgcccagcacctgaactcctggggggaccgtcagtcttcctcttccccccaaaacccaaggacaccctcatgatctcccggacccctgaggtcacatgcgtggtggtggacgtgagccacgaagaccctgaggtcaagttcaactggtacgtggacggcgtggaggtgcataatgccaagacaaagccgcgggaggagcagtacaacagcacgtaccgtgtggtcagcgtcctcaccgtcctgcaccaggactggctgaatggcaaggagtacaagtgcaaggtctccaacaaagccctcccagcccccatcgagaaaaccatctccaaagccaaagggcagccccgagaaccacaggtgtacaccctgcccccatcccgggatgagctgaccaagaaccaggtcagcctgacctgcctggtcaaaggcttctatcccagcgacatcgccgtggagtgggagagcaatgggcagccggagaacaactacaagaccacgcctcccgtgctggactccgacggctccttcttcctctacagcaagctcaccgtggacaagagcaggtggcagcaggggaacgtcttctcatgctccgtgatgcatgaggctctgcacaaccactacacacagaagagcctctccctgtctccgggtaaatga

SEQ ID NO: 49 - protein, 476 aa, Artificial Sequence
  Synthetic
AVTLDESGGGLQTPGGALSLVCKASGFTFSSNAMGWVRQAPGKGLEWVAGIDDDGSGTRYAPAVKGRATISRDNGQSTLRLQLNNLRAEDTGTYYCAKLEVTCEPGTTFKDKCNTCRCGSDGKSAFCTRKLCYQAWGHGTEVIVSSASTKGPSVFPLAPSSKSTSGGTAALGCLVKDYFPEPVTVSWNSGALTSGVHTFPAVLQSSGLYSLSSVVTVPSSSLGTQTYICNVNHKPSNTKVDKKVEPKSCDKTHTCPPCPAPELLGGPSVFLFPPKPKDTLMISRTPEVTCVVVDVSHEDPEVKFNWYVDGVEVHNAKTKPREEQYNSTYRVVSVLTVLHQDWLNGKEYKCKVSNKALPAPIEKTISKAKGQPREPQVYTLPPSRDELTKNQVSLTCLVKGFYPSDIAVEWESNGQPENNYKTTPPVLDSDGSFFLYSKLTVDKSRWQQGNVFSCSVMHEALHNHYTQKSLSLSPGK

SEQ ID NO: 50 - DNA, 1479 bp, Artificial Sequence
  Synthetic
atggagttcggcctgagctggctgttcctggtggccatccttaagggcgtgcagtgcgccgtgacgttggacgagtccgggggcggcctccagacgcccgggggagcgctcagcctcgtctgcaaggcctccgggttcaccttcagcagtaacgccatgggttgggtgcgacaggcgcccggcaaggggctggagtgggtcgctggtattgatgatgatggtagtggcacaagatacgcgccggcggtgaagggccgtgccaccatctcgagggacaacgggcagagcacactgaggctgcagctgaacaacctcagggctgaggacaccggcacctactactgcgccaaaacatgtgaacccggtacgacgtttaaggataagtgcaacacatgtaggtgcggtagcgacggcaaatcagcgttctgtacccggaaattgtgctaccaggcatggggccacgggaccgaagtcatcgtctcctccgctagcaccaagggcccatcggtcttccccctggcaccctcctccaagagcacctctgggggcacagcggccctgggctgcctggtcaaggactacttccccgaaccggtgacggtgtcgtggaactcaggcgccctgaccagcggcgtgcacaccttcccggctgtcctacagtcctcaggactctactccctcagcagcgtggtgaccgtgccctccagcagcttgggcacccagacctacatctgcaacgtgaatcacaagcccagcaacaccaaggtggacaagaaagttgagcccaaatcttgtgacaaaactcacacatgcccaccgtgcccagcacctgaactcctggggggaccgtcagtcttcctcttccccccaaaacccaaggacaccctcatgatctcccggacccctgaggtcacatgcgtggtggtggacgtgagccacgaagaccctgaggtcaagttcaactggtacgtggacggcgtggaggtgcataatgccaagacaaagccgcgggaggagcagtacaacagcacgtaccgtgtggtcagcgtcctcaccgtcctgcaccaggactggctgaatggcaaggagtacaagtgcaaggtctccaacaaagccctcccagcccccatcgagaaaaccatctccaaagccaaagggcagccccgagaaccacaggtgtacaccctgcccccatcccgggatgagctgaccaagaaccaggtcagcctgacctgcctggtcaaaggcttctatcccagcgacatcgccgtggagtgggagagcaatgggcagccggagaacaactacaagaccacgcctcccgtgctggactccgacggctccttcttcctctacagcaagctcaccgtggacaagagcaggtggcagcaggggaacgtcttctcatgctccgtgatgcatgaggctctgcacaaccactacacacagaagagcctctccctgtctccgggtaaatga

SEQ ID NO: 51 - protein, 473 aa, Artificial Sequence
  Synthetic
AVTLDESGGGLQTPGGALSLVCKASGFTFSSNAMGWVRQAPGKGLEWVAGIDDDGSGTRYAPAVKGRATISRDNGQSTLRLQLNNLRAEDTGTYYCAKTCEPGTTFKDKCNTCRCGSDGKSAFCTRKLCYQAWGHGTEVIVSSASTKGPSVFPLAPSSKSTSGGTAALGCLVKDYFPEPVTVSWNSGALTSGVHTFPAVLQSSGLYSLSSVVTVPSSSLGTQTYICNVNHKPSNTKVDKKVEPKSCDKTHTCPPCPAPELLGGPSVFLFPPKPKDTLMISRTPEVTCVVVDVSHEDPEVKFNWYVDGVEVHNAKTKPREEQYNSTYRVVSVLTVLHQDWLNGKEYKCKVSNKALPAPIEKTISKAKGQPREPQVYTLPPSRDELTKNQVSLTCLVKGFYPSDIAVEWESNGQPENNYKTTPPVLDSDGSFFLYSKLTVDKSRWQQGNVFSCSVMHEALHNHYTQKSLSLSPGK

SEQ ID NO: 52 - DNA, 1440 bp, Artificial Sequence
  Synthetic
atggagttcggcctgagctggctgttcctggtggccatccttaagggcgtgcagtgcgccgtgacgttggacgagtccgggggcggcctccagacgcccgggggagcgctcagcctcgtctgcaaggcctccgggttcaccttcagcagtaacgccatgggttgggtgcgacaggcgcccggcaaggggctggagtgggtcgctggtattgatgatgatggtagtggcacaagatacgcgccggcggtgaagggccgtgccaccatctcgagggacaacgggcagagcacactgaggctgcagctgaacaacctcagggctgaggacaccggcacctactactgcgccaaaacatgtaggtgcggtagcgacggcaaatcagcgttctgtacccggaaattgtgctaccaggcatggggccacgggaccgaagtcatcgtctcctccgctagcaccaagggcccatcggtcttccccctggcaccctcctccaagagcacctctgggggcacagcggccctgggctgcctggtcaaggactacttccccgaaccggtgacggtgtcgtggaactcaggcgccctgaccagcggcgtgcacaccttcccggctgtcctacagtcctcaggactctactccctcagcagcgtggtgaccgtgccctccagcagcttgggcacccagacctacatctgcaacgtgaatcacaagcccagcaacaccaaggtggacaagaaagttgagcccaaatcttgtgacaaaactcacacatgcccaccgtgcccagcacctgaactcctggggggaccgtcagtcttcctcttccccccaaaacccaaggacaccctcatgatctcccggacccctgaggtcacatgcgtggtggtggacgtgagccacgaagaccctgaggtcaagttcaactggtacgtggacggcgtggaggtgcataatgccaagacaaagccgcgggaggagcagtacaacagcacgtaccgtgtggtcagcgtcctcaccgtcctgcaccaggactggctgaatggcaaggagtacaagtgcaaggtctccaacaaagccctcccagcccccatcgagaaaaccatctccaaagccaaagggcagccccgagaaccacaggtgtacaccctgcccccatcccgggatgagctgaccaagaaccaggtcagcctgacctgcctggtcaaaggcttctatcccagcgacatcgccgtggagtgggagagcaatgggcagccggagaacaactacaagaccacgcctcccgtgctggactccgacggctccttcttcctctacagcaagctcaccgtggacaagagcaggtggcagcaggggaacgtcttctcatgctccgtgatgcatgaggctctgcacaaccactacacacagaagagcctctccctgtctccgggtaaatga

SEQ ID NO: 53 - protein, 460 aa, Artificial Sequence
  Synthetic
AVTLDESGGGLQTPGGALSLVCKASGFTFSSNAMGWVRQAPGKGLEWVAGIDDDGSGTRYAPAVKGRATISRDNGQSTLRLQLNNLRAEDTGTYYCAKTCRCGSDGKSAFCTRKLCYQAWGHGTEVIVSSASTKGPSVFPLAPSSKSTSGGTAALGCLVKDYFPEPVTVSWNSGALTSGVHTFPAVLQSSGLYSLSSVVTVPSSSLGTQTYICNVNHKPSNTKVDKKVEPKSCDKTHTCPPCPAPELLGGPSVFLFPPKPKDTLMISRTPEVTCVVVDVSHEDPEVKFNWYVDGVEVHNAKTKPREEQYNSTYRVVSVLTVLHQDWLNGKEYKCKVSNKALPAPIEKTISKAKGQPREPQVYTLPPSRDELTKNQVSLTCLVKGFYPSDIAVEWESNGQPENNYKTTPPVLDSDGSFFLYSKLTVDKSRWQQGNVFSCSVMHEALHNHYTQKSLSLSPGK

SEQ ID NO: 54 - DNA, 1527 bp, Artificial Sequence
  Synthetic
atggagttcggcctgagctggctgttcctggtggccatccttaagggcgtgcagtgcgccgtgacgttggacgagtccgggggcggcctccagacgcccgggggagcgctcagcctcgtctgcaaggcctccgggttcaccttcagcagtaacgccatgggttgggtgcgacaggcgcccggcaaggggctggagtgggtcgctggtattgatgatgatggtagtggcacaagatacgcgccggcggtgaagggccgtgccaccatctcgagggacaacgggcagagcacactgaggctgcagctgaacaacctcagggctgaggacaccggcacctactactgcgccaaactcgaggtgacatgtgaacccggtacgacgtttaaggataagtgcaacacatgtaggtgcggtagcgacggcaaatcagcgttctgtacccggaaattgtgctaccagggaactggaggagggtcggggtcctcgtcatatatcgacgcatggggccacgggaccgaagtcatcgtctcctccgctagcaccaagggcccatcggtcttccccctggcaccctcctccaagagcacctctgggggcacagcggccctgggctgcctggtcaaggactacttccccgaaccggtgacggtgtcgtggaactcaggcgccctgaccagcggcgtgcacaccttcccggctgtcctacagtcctcaggactctactccctcagcagcgtggtgaccgtgccctccagcagcttgggcacccagacctacatctgcaacgtgaatcacaagcccagcaacaccaaggtggacaagaaagttgagcccaaatcttgtgacaaaactcacacatgcccaccgtgcccagcacctgaactcctggggggaccgtcagtcttcctcttccccccaaaacccaaggacaccctcatgatctcccggacccctgaggtcacatgcgtggtggtggacgtgagccacgaagaccctgaggtcaagttcaactggtacgtggacggcgtggaggtgcataatgccaagacaaagccgcgggaggagcagtacaacagcacgtaccgtgtggtcagcgtcctcaccgtcctgcaccaggactggctgaatggcaaggagtacaagtgcaaggtctccaacaaagccctcccagcccccatcgagaaaaccatctccaaagccaaagggcagccccgagaaccacaggtgtacaccctgcccccatcccgggatgagctgaccaagaaccaggtcagcctgacctgcctggtcaaaggcttctatcccagcgacatcgccgtggagtgggagagcaatgggcagccggagaacaactacaagaccacgcctcccgtgctggactccgacggctccttcttcctctacagcaagctcaccgtggacaagagcaggtggcagcaggggaacgtcttctcatgctccgtgatgcatgaggctctgcacaaccactacacacagaagagcctctccctgtctccgggtaaatga

SEQ ID NO: 55 - protein, 489 aa, Artificial Sequence
  Synthetic
AVTLDESGGGLQTPGGALSLVCKASGFTFSSNAMGWVRQAPGKGLEWVAGIDDDGSGTRYAPAVKGRATISRDNGQSTLRLQLNNLRAEDTGTYYCAKLEVTCEPGTTFKDKCNTCRCGSDGKSAFCTRKLCYQGTGGGSGSSSYIDAWGHGTEVIVSSASTKGPSVFPLAPSSKSTSGGTAALGCLVKDYFPEPVTVSWNSGALTSGVHTFPAVLQSSGLYSLSSVVTVPSSSLGTQTYICNVNHKPSNTKVDKKVEPKSCDKTHTCPPCPAPELLGGPSVFLFPPKPKDTLMISRTPEVTCVVVDVSHEDPEVKFNWYVDGVEVHNAKTKPREEQYNSTYRVVSVLTVLHQDWLNGKEYKCKVSNKALPAPIEKTISKAKGQPREPQVYTLPPSRDELTKNQVSLTCLVKGFYPSDIAVEWESNGQPENNYKTTPPVLDSDGSFFLYSKLTVDKSRWQQGNVFSCSVMHEALHNHYTQKSLSLSPGK

SEQ ID NO: 56 - DNA, 1557 bp, Artificial Sequence
  Synthetic
atggagttcggcctgagctggctgttcctggtggccatccttaagggcgtgcagtgcgccgtgacgttggacgagtccgggggcggcctccagacgcccgggggagcgctcagcctcgtctgcaaggcctccgggttcaccttcagcagtaacgccatgggttgggtgcgacaggcgcccggcaaggggctggagtgggtcgctggtattgatgatgatggtagtggcacaagatacgcgccggcggtgaagggccgtgccaccatctcgagggacaacgggcagagcacactgaggctgcagctgaacaacctcagggctgaggacaccggcacctactactgcgccaaaggcaccggtggagggtcgggatccagctcactcgaggtgacatgtgaacccggtacgacgtttaaggataagtgcaacacatgtaggtgcggtagcgacggcaaatcagcgttctgtacccggaaattgtgctaccagggaactggaggagggtcggggtcctcgtcatatatcgacgcatggggccacgggaccgaagtcatcgtctcctccgctagcaccaagggcccatcggtcttccccctggcaccctcctccaagagcacctctgggggcacagcggccctgggctgcctggtcaaggactacttccccgaaccggtgacggtgtcgtggaactcaggcgccctgaccagcggcgtgcacaccttcccggctgtcctacagtcctcaggactctactccctcagcagcgtggtgaccgtgccctccagcagcttgggcacccagacctacatctgcaacgtgaatcacaagcccagcaacaccaaggtggacaagaaagttgagcccaaatcttgtgacaaaactcacacatgcccaccgtgcccagcacctgaactcctggggggaccgtcagtcttcctcttccccccaaaacccaaggacaccctcatgatctcccggacccctgaggtcacatgcgtggtggtggacgtgagccacgaagaccctgaggtcaagttcaactggtacgtggacggcgtggaggtgcataatgccaagacaaagccgcgggaggagcagtacaacagcacgtaccgtgtggtcagcgtcctcaccgtcctgcaccaggactggctgaatggcaaggagtacaagtgcaaggtctccaacaaagccctcccagcccccatcgagaaaaccatctccaaagccaaagggcagccccgagaaccacaggtgtacaccctgcccccatcccgggatgagctgaccaagaaccaggtcagcctgacctgcctggtcaaaggcttctatcccagcgacatcgccgtggagtgggagagcaatgggcagccggagaacaactacaagaccacgcctcccgtgctggactccgacggctccttcttcctctacagcaagctcaccgtggacaagagcaggtggcagcaggggaacgtcttctcatgctccgtgatgcatgaggctctgcacaaccactacacacagaagagcctctccctgtctccgggtaaatga

SEQ ID NO: 57 - protein, 499 aa, Artificial Sequence
  Synthetic
AVTLDESGGGLQTPGGALSLVCKASGFTFSSNAMGWVRQAPGKGLEWVAGIDDDGSGTRYAPAVKGRATISRDNGQSTLRLQLNNLRAEDTGTYYCAKGTGGGSGSSSLEVTCEPGTTFKDKCNTCRCGSDGKSAFCTRKLCYQGTGGGSGSSSYIDAWGHGTEVIVSSASTKGPSVFPLAPSSKSTSGGTAALGCLVKDYFPEPVTVSWNSGALTSGVHTFPAVLQSSGLYSLSSVVTVPSSSLGTQTYICNVNHKPSNTKVDKKVEPKSCDKTHTCPPCPAPELLGGPSVFLFPPKPKDTLMISRTPEVTCVVVDVSHEDPEVKFNWYVDGVEVHNAKTKPREEQYNSTYRVVSVLTVLHQDWLNGKEYKCKVSNKALPAPIEKTISKAKGQPREPQVYTLPPSRDELTKNQVSLTCLVKGFYPSDIAVEWESNGQPENNYKTTPPVLDSDGSFFLYSKLTVDKSRWQQGNVFSCSVMHEALHNHYTQKSLSLSPGK

SEQ ID NO: 58 - DNA, 1545 bp, Artificial Sequence
  Synthetic
atggagttcggcctgagctggctgttcctggtggccatccttaagggcgtgcagtgcgccgtgacgttggacgagtccgggggcggcctccagacgcccgggggagcgctcagcctcgtctgcaaggcctccgggttcaccttcagcagtaacgccatgggttgggtgcgacaggcgcccggcaaggggctggagtgggtcgctggtattgatgatgatggtagtggcacaagatacgcgccggcggtgaagggccgtgccaccatctcgagggacaacgggcagagcacactgaggctgcagctgaacaacctcagggctgaggacaccggcacctactactgcgccaaagccgctggtggtagtggtctcgaggtgacatgtgaacccggtacgacgtttaaggataagtgcaacacatgtaggtgcggtagcgacggcaaatcagcgttctgtacccggaaattgtgctaccagggaactggaggagggtcggggtcctcgtcatatatcgacgcatggggccacgggaccgaagtcatcgtctcctccgctagcaccaagggcccatcggtcttccccctggcaccctcctccaagagcacctctgggggcacagcggccctgggctgcctggtcaaggactacttccccgaaccggtgacggtgtcgtggaactcaggcgccctgaccagcggcgtgcacaccttcccggctgtcctacagtcctcaggactctactccctcagcagcgtggtgaccgtgccctccagcagcttgggcacccagacctacatctgcaacgtgaatcacaagcccagcaacaccaaggtggacaagaaagttgagcccaaatcttgtgacaaaactcacacatgcccaccgtgcccagcacctgaactcctggggggaccgtcagtcttcctcttccccccaaaacccaaggacaccctcatgatctcccggacccctgaggtcacatgcgtggtggtggacgtgagccacgaagaccctgaggtcaagttcaactggtacgtggacggcgtggaggtgcataatgccaagacaaagccgcgggaggagcagtacaacagcacgtaccgtgtggtcagcgtcctcaccgtcctgcaccaggactggctgaatggcaaggagtacaagtgcaaggtctccaacaaagccctcccagcccccatcgagaaaaccatctccaaagccaaagggcagccccgagaaccacaggtgtacaccctgcccccatcccgggatgagctgaccaagaaccaggtcagcctgacctgcctggtcaaaggcttctatcccagcgacatcgccgtggagtgggagagcaatgggcagccggagaacaactacaagaccacgcctcccgtgctggactccgacggctccttcttcctctacagcaagctcaccgtggacaagagcaggtggcagcaggggaacgtcttctcatgctccgtgatgcatgaggctctgcacaaccactacacacagaagagcctctccctgtctccgggtaaatga

SEQ ID NO: 59 - protein, 495 aa, Artificial Sequence
  Synthetic
AVTLDESGGGLQTPGGALSLVCKASGFTFSSNAMGWVRQAPGKGLEWVAGIDDDGSGTRYAPAVKGRATISRDNGQSTLRLQLNNLRAEDTGTYYCAKAAGGSGLEVTCEPGTTFKDKCNTCRCGSDGKSAFCTRKLCYQGTGGGSGSSSYIDAWGHGTEVIVSSASTKGPSVFPLAPSSKSTSGGTAALGCLVKDYFPEPVTVSWNSGALTSGVHTFPAVLQSSGLYSLSSVVTVPSSSLGTQTYICNVNHKPSNTKVDKKVEPKSCDKTHTCPPCPAPELLGGPSVFLFPPKPKDTLMISRTPEVTCVVVDVSHEDPEVKFNWYVDGVEVHNAKTKPREEQYNSTYRVVSVLTVLHQDWLNGKEYKCKVSNKALPAPIEKTISKAKGQPREPQVYTLPPSRDELTKNQVSLTCLVKGFYPSDIAVEWESNGQPENNYKTTPPVLDSDGSFFLYSKLTVDKSRWQQGNVFSCSVMHEALHNHYTQKSLSLSPGK

SEQ ID NO: 60 - DNA, 1509 bp, Artificial Sequence
  Synthetic
atggagttcggcctgagctggctgttcctggtggccatccttaagggcgtgcagtgcgccgtgacgttggacgagtccgggggcggcctccagacgcccgggggagcgctcagcctcgtctgcaaggcctccgggttcaccttcagcagtaacgccatgggttgggtgcgacaggcgcccggcaaggggctggagtgggtcgctggtattgatgatgatggtagtggcacaagatacgcgccggcggtgaagggccgtgccaccatctcgagggacaacgggcagagcacactgaggctgcagctgaacaacctcagggctgaggacaccggcacctactactgcgccaaactcgaggtgacatgtgaacccggtacgacgtttaaggataagtgcaacacatgtaggtgcggtagcgacggcaaatcagcgttctgtacccggaaattgtgctaccagggtagtggtgcttatatcgacgcatggggccacgggaccgaagtcatcgtctcctccgctagcaccaagggcccatcggtcttccccctggcaccctcctccaagagcacctctgggggcacagcggccctgggctgcctggtcaaggactacttccccgaaccggtgacggtgtcgtggaactcaggcgccctgaccagcggcgtgcacaccttcccggctgtcctacagtcctcaggactctactccctcagcagcgtggtgaccgtgccctccagcagcttgggcacccagacctacatctgcaacgtgaatcacaagcccagcaacaccaaggtggacaagaaagttgagcccaaatcttgtgacaaaactcacacatgcccaccgtgcccagcacctgaactcctggggggaccgtcagtcttcctcttccccccaaaacccaaggacaccctcatgatctcccggacccctgaggtcacatgcgtggtggtggacgtgagccacgaagaccctgaggtcaagttcaactggtacgtggacggcgtggaggtgcataatgccaagacaaagccgcgggaggagcagtacaacagcacgtaccgtgtggtcagcgtcctcaccgtcctgcaccaggactggctgaatggcaaggagtacaagtgcaaggtctccaacaaagccctcccagcccccatcgagaaaaccatctccaaagccaaagggcagccccgagaaccacaggtgtacaccctgcccccatcccgggatgagctgaccaagaaccaggtcagcctgacctgcctggtcaaaggcttctatcccagcgacatcgccgtggagtgggagagcaatgggcagccggagaacaactacaagaccacgcctcccgtgctggactccgacggctccttcttcctctacagcaagctcaccgtggacaagagcaggtggcagcaggggaacgtcttctcatgctccgtgatgcatgaggctctgcacaaccactacacacagaagagcctctccctgtctccgggtaaatga

SEQ ID NO: 61 - protein, 493 aa, Artificial Sequence
  Synthetic
AVTLDESGGGLQTPGGALSLVCKASGFTFSSNAMGWVRQAPGKGLEWVAGIDDDGSGTRYAPAVKGRATISRDNGQSTLRLQLNNLRAEDTGTYYCAKGTGGGSGSSSLEVTCEPGTTFKDKCNTCRCGSDGKSAFCTRKLCYQGSGAYIDAWGHGTEVIVSSASTKGPSVFPLAPSSKSTSGGTAALGCLVKDYFPEPVTVSWNSGALTSGVHTFPAVLQSSGLYSLSSVVTVPSSSLGTQTYICNVNHKPSNTKVDKKVEPKSCDKTHTCPPCPAPELLGGPSVFLFPPKPKDTLMISRTPEVTCVVVDVSHEDPEVKFNWYVDGVEVHNAKTKPREEQYNSTYRVVSVLTVLHQDWLNGKEYKCKVSNKALPAPIEKTISKAKGQPREPQVYTLPPSRDELTKNQVSLTCLVKGFYPSDIAVEWESNGQPENNYKTTPPVLDSDGSFFLYSKLTVDKSRWQQGNVFSCSVMHEALHNHYTQKSLSLSPGK

SEQ ID NO: 62 - DNA, 1527 bp, Artificial Sequence
  Synthetic
atggagttcggcctgagctggctgttcctggtggccatccttaagggcgtgcagtgcgccgtgacgttggacgagtccgggggcggcctccagacgcccgggggagcgctcagcctcgtctgcaaggcctccgggttcaccttcagcagtaacgccatgggttgggtgcgacaggcgcccggcaaggggctggagtgggtcgctggtattgatgatgatggtagtggcacaagatacgcgccggcggtgaagggccgtgccaccatctcgagggacaacgggcagagcacactgaggctgcagctgaacaacctcagggctgaggacaccggcacctactactgcgccaaagccgctggtggtagtggtctcgaggtgacatgtgaacccggtacgacgtttaaggataagtgcaacacatgtaggtgcggtagcgacggcaaatcagcgttctgtacccggaaattgtgctaccagggtagtggtgcttatatcgacgcatggggccacgggaccgaagtcatcgtctcctccgctagcaccaagggcccatcggtcttccccctggcaccctcctccaagagcacctctgggggcacagcggccctgggctgcctggtcaaggactacttccccgaaccggtgacggtgtcgtggaactcaggcgccctgaccagcggcgtgcacaccttcccggctgtcctacagtcctcaggactctactccctcagcagcgtggtgaccgtgccctccagcagcttgggcacccagacctacatctgcaacgtgaatcacaagcccagcaacaccaaggtggacaagaaagttgagcccaaatcttgtgacaaaactcacacatgcccaccgtgcccagcacctgaactcctggggggaccgtcagtcttcctcttccccccaaaacccaaggacaccctcatgatctcccggacccctgaggtcacatgcgtggtggtggacgtgagccacgaagaccctgaggtcaagttcaactggtacgtggacggcgtggaggtgcataatgccaagacaaagccgcgggaggagcagtacaacagcacgtaccgtgtggtcagcgtcctcaccgtcctgcaccaggactggctgaatggcaaggagtacaagtgcaaggtctccaacaaagccctcccagcccccatcgagaaaaccatctccaaagccaaagggcagccccgagaaccacaggtgtacaccctgcccccatcccgggatgagctgaccaagaaccaggtcagcctgacctgcctggtcaaaggcttctatcccagcgacatcgccgtggagtgggagagcaatgggcagccggagaacaactacaagaccacgcctcccgtgctggactccgacggctccttcttcctctacagcaagctcaccgtggacaagagcaggtggcagcaggggaacgtcttctcatgctccgtgatgcatgaggctctgcacaaccactacacacagaagagcctctccctgtctccgggtaaatga

SEQ ID NO: 63 - protein, 489 aa, Artificial Sequence
  Synthetic
AVTLDESGGGLQTPGGALSLVCKASGFTFSSNAMGWVRQAPGKGLEWVAGIDDDGSGTRYAPAVKGRATISRDNGQSTLRLQLNNLRAEDTGTYYCAKAAGGSGLEVTCEPGTTFKDKCNTCRCGSDGKSAFCTRKLCYQGSGAYIDAWGHGTEVIVSSASTKGPSVFPLAPSSKSTSGGTAALGCLVKDYFPEPVTVSWNSGALTSGVHTFPAVLQSSGLYSLSSVVTVPSSSLGTQTYICNVNHKPSNTKVDKKVEPKSCDKTHTCPPCPAPELLGGPSVFLFPPKPKDTLMISRTPEVTCVVVDVSHEDPEVKFNWYVDGVEVHNAKTKPREEQYNSTYRVVSVLTVLHQDWLNGKEYKCKVSNKALPAPIEKTISKAKGQPREPQVYTLPPSRDELTKNQVSLTCLVKGFYPSDIAVEWESNGQPENNYKTTPPVLDSDGSFFLYSKLTVDKSRWQQGNVFSCSVMHEALHNHYTQKSLSLSPGK

SEQ ID NO: 64 - DNA, 1539 bp, Artificial Sequence
  Synthetic
atggagttcggcctgagctggctgttcctggtggccatccttaagggcgtgcagtgcgccgtgacgttggacgagtccgggggcggcctccagacgcccgggggagcgctcagcctcgtctgcaaggcctccgggttcaccttcagcagtaacgccatgggttgggtgcgacaggcgcccggcaaggggctggagtgggtcgctggtattgatgatgatggtagtggcacaagatacgcgccggcggtgaagggccgtgccaccatctcgagggacaacgggcagagcacactgaggctgcagctgaacaacctcagggctgaggacaccggcacctactactgcgccaaagccgctggtggtagtggtggtagtggtgctctcgaggtgacatgtgaacccggtacgacgtttaaggataagtgcaacacatgtaggtgcggtagcgacggcaaatcagcgttctgtacccggaaattgtgctaccagggtagtggtgcttatatcgacgcatggggccacgggaccgaagtcatcgtctcctccgctagcaccaagggcccatcggtcttccccctggcaccctcctccaagagcacctctgggggcacagcggccctgggctgcctggtcaaggactacttccccgaaccggtgacggtgtcgtggaactcaggcgccctgaccagcggcgtgcacaccttcccggctgtcctacagtcctcaggactctactccctcagcagcgtggtgaccgtgccctccagcagcttgggcacccagacctacatctgcaacgtgaatcacaagcccagcaacaccaaggtggacaagaaagttgagcccaaatcttgtgacaaaactcacacatgcccaccgtgcccagcacctgaactcctggggggaccgtcagtcttcctcttccccccaaaacccaaggacaccctcatgatctcccggacccctgaggtcacatgcgtggtggtggacgtgagccacgaagaccctgaggtcaagttcaactggtacgtggacggcgtggaggtgcataatgccaagacaaagccgcgggaggagcagtacaacagcacgtaccgtgtggtcagcgtcctcaccgtcctgcaccaggactggctgaatggcaaggagtacaagtgcaaggtctccaacaaagccctcccagcccccatcgagaaaaccatctccaaagccaaagggcagccccgagaaccacaggtgtacaccctgcccccatcccgggatgagctgaccaagaaccaggtcagcctgacctgcctggtcaaaggcttctatcccagcgacatcgccgtggagtgggagagcaatgggcagccggagaacaactacaagaccacgcctcccgtgctggactccgacggctccttcttcctctacagcaagctcaccgtggacaagagcaggtggcagcaggggaacgtcttctcatgctccgtgatgcatgaggctctgcacaaccactacacacagaagagcctctccctgtctccgggtaaatga

SEQ ID NO: 65 - protein, 493 aa, Artificial Sequence
  Synthetic
AVTLDESGGGLQTPGGALSLVCKASGFTFSSNAMGWVRQAPGKGLEWVAGIDDDGSGTRYAPAVKGRATISRDNGQSTLRLQLNNLRAEDTGTYYCAKAAGGSGGSGALEVTCEPGTTFKDKCNTCRCGSDGKSAFCTRKLCYQGSGAYIDAWGHGTEVIVSSASTKGPSVFPLAPSSKSTSGGTAALGCLVKDYFPEPVTVSWNSGALTSGVHTFPAVLQSSGLYSLSSVVTVPSSSLGTQTYICNVNHKPSNTKVDKKVEPKSCDKTHTCPPCPAPELLGGPSVFLFPPKPKDTLMISRTPEVTCVVVDVSHEDPEVKFNWYVDGVEVHNAKTKPREEQYNSTYRVVSVLTVLHQDWLNGKEYKCKVSNKALPAPIEKTISKAKGQPREPQVYTLPPSRDELTKNQVSLTCLVKGFYPSDIAVEWESNGQPENNYKTTPPVLDSDGSFFLYSKLTVDKSRWQQGNVFSCSVMHEALHNHYTQKSLSLSPGK

SEQ ID NO: 66 - DNA, 1527 bp, Artificial Sequence
  Synthetic
atggagttcggcctgagctggctgttcctggtggccatccttaagggcgtgcagtgcgccgtgacgttggacgagtccgggggcggcctccagacgcccgggggagcgctcagcctcgtctgcaaggcctccgggttcaccttcagcagtaacgccatgggttgggtgcgacaggcgcccggcaaggggctggagtgggtcgctggtattgatgatgatggtagtggcacaagatacgcgccggcggtgaagggccgtgccaccatctcgagggacaacgggcagagcacactgaggctgcagctgaacaacctcagggctgaggacaccggcacctactactgcgccaaactcgaggtgacatgtgaacccggtacgacgtttaaggataagtgcaacacatgtaggtgcggtagcgacggcaaatcagcgttctgtacccggaaattgtgctaccaggccgctggtggtagtggtggtagtggtgcttatatcgacgcatggggccacgggaccgaagtcatcgtctcctccgctagcaccaagggcccatcggtcttccccctggcaccctcctccaagagcacctctgggggcacagcggccctgggctgcctggtcaaggactacttccccgaaccggtgacggtgtcgtggaactcaggcgccctgaccagcggcgtgcacaccttcccggctgtcctacagtcctcaggactctactccctcagcagcgtggtgaccgtgccctccagcagcttgggcacccagacctacatctgcaacgtgaatcacaagcccagcaacaccaaggtggacaagaaagttgagcccaaatcttgtgacaaaactcacacatgcccaccgtgcccagcacctgaactcctggggggaccgtcagtcttcctcttccccccaaaacccaaggacaccctcatgatctcccggacccctgaggtcacatgcgtggtggtggacgtgagccacgaagaccctgaggtcaagttcaactggtacgtggacggcgtggaggtgcataatgccaagacaaagccgcgggaggagcagtacaacagcacgtaccgtgtggtcagcgtcctcaccgtcctgcaccaggactggctgaatggcaaggagtacaagtgcaaggtctccaacaaagccctcccagcccccatcgagaaaaccatctccaaagccaaagggcagccccgagaaccacaggtgtacaccctgcccccatcccgggatgagctgaccaagaaccaggtcagcctgacctgcctggtcaaaggcttctatcccagcgacatcgccgtggagtgggagagcaatgggcagccggagaacaactacaagaccacgcctcccgtgctggactccgacggctccttcttcctctacagcaagctcaccgtggacaagagcaggtggcagcaggggaacgtcttctcatgctccgtgatgcatgaggctctgcacaaccactacacacagaagagcctctccctgtctccgggtaaatga

SEQ ID NO: 67 - protein, 489 aa, Artificial Sequence
  Synthetic
AVTLDESGGGLQTPGGALSLVCKASGFTFSSNAMGWVRQAPGKGLEWVAGIDDDGSGTRYAPAVKGRATISRDNGQSTLRLQLNNLRAEDTGTYYCAKLEVTCEPGTTFKDKCNTCRCGSDGKSAFCTRKLCYQAAGGSGGSGAYIDAWGHGTEVIVSSASTKGPSVFPLAPSSKSTSGGTAALGCLVKDYFPEPVTVSWNSGALTSGVHTFPAVLQSSGLYSLSSVVTVPSSSLGTQTYICNVNHKPSNTKVDKKVEPKSCDKTHTCPPCPAPELLGGPSVFLFPPKPKDTLMISRTPEVTCVVVDVSHEDPEVKFNWYVDGVEVHNAKTKPREEQYNSTYRVVSVLTVLHQDWLNGKEYKCKVSNKALPAPIEKTISKAKGQPREPQVYTLPPSRDELTKNQVSLTCLVKGFYPSDIAVEWESNGQPENNYKTTPPVLDSDGSFFLYSKLTVDKSRWQQGNVFSCSVMHEALHNHYTQKSLSLSPGK

SEQ ID NO: 68 - DNA, 1557 bp, Artificial Sequence
  Synthetic
atggagttcggcctgagctggctgttcctggtggccatccttaagggcgtgcagtgcgccgtgacgttggacgagtccgggggcggcctccagacgcccgggggagcgctcagcctcgtctgcaaggcctccgggttcaccttcagcagtaacgccatgggttgggtgcgacaggcgcccggcaaggggctggagtgggtcgctggtattgatgatgatggtagtggcacaagatacgcgccggcggtgaagggccgtgccaccatctcgagggacaacgggcagagcacactgaggctgcagctgaacaacctcagggctgaggacaccggcacctactactgcgccaaaggcaccggtggagggtcgggatccagctcactcgaggtgacatgtgaacccggtacgacgtttaaggataagtgcaacacatgtaggtgcggtagcgacggcaaatcagcgttctgtacccggaaattgtgctaccaggccgctggtggtagtggtggtagtggtgcttatatcgacgcatggggccacgggaccgaagtcatcgtctcctccgctagcaccaagggcccatcggtcttccccctggcaccctcctccaagagcacctctgggggcacagcggccctgggctgcctggtcaaggactacttccccgaaccggtgacggtgtcgtggaactcaggcgccctgaccagcggcgtgcacaccttcccggctgtcctacagtcctcaggactctactccctcagcagcgtggtgaccgtgccctccagcagcttgggcacccagacctacatctgcaacgtgaatcacaagcccagcaacaccaaggtggacaagaaagttgagcccaaatcttgtgacaaaactcacacatgcccaccgtgcccagcacctgaactcctggggggaccgtcagtcttcctcttccccccaaaacccaaggacaccctcatgatctcccggacccctgaggtcacatgcgtggtggtggacgtgagccacgaagaccctgaggtcaagttcaactggtacgtggacggcgtggaggtgcataatgccaagacaaagccgcgggaggagcagtacaacagcacgtaccgtgtggtcagcgtcctcaccgtcctgcaccaggactggctgaatggcaaggagtacaagtgcaaggtctccaacaaagccctcccagcccccatcgagaaaaccatctccaaagccaaagggcagccccgagaaccacaggtgtacaccctgcccccatcccgggatgagctgaccaagaaccaggtcagcctgacctgcctggtcaaaggcttctatcccagcgacatcgccgtggagtgggagagcaatgggcagccggagaacaactacaagaccacgcctcccgtgctggactccgacggctccttcttcctctacagcaagctcaccgtggacaagagcaggtggcagcaggggaacgtcttctcatgctccgtgatgcatgaggctctgcacaaccactacacacagaagagcctctccctgtctccgggtaaatga

SEQ ID NO: 69 - protein, 499 aa, Artificial Sequence
  Synthetic
AVTLDESGGGLQTPGGALSLVCKASGFTFSSNAMGWVRQAPGKGLEWVAGIDDDGSGTRYAPAVKGRATISRDNGQSTLRLQLNNLRAEDTGTYYCAKGTGGGSGSSSLEVTCEPGTTFKDKCNTCRCGSDGKSAFCTRKLCYQAAGGSGGSGAYIDAWGHGTEVIVSSASTKGPSVFPLAPSSKSTSGGTAALGCLVKDYFPEPVTVSWNSGALTSGVHTFPAVLQSSGLYSLSSVVTVPSSSLGTQTYICNVNHKPSNTKVDKKVEPKSCDKTHTCPPCPAPELLGGPSVFLFPPKPKDTLMISRTPEVTCVVVDVSHEDPEVKFNWYVDGVEVHNAKTKPREEQYNSTYRVVSVLTVLHQDWLNGKEYKCKVSNKALPAPIEKTISKAKGQPREPQVYTLPPSRDELTKNQVSLTCLVKGFYPSDIAVEWESNGQPENNYKTTPPVLDSDGSFFLYSKLTVDKSRWQQGNVFSCSVMHEALHNHYTQKSLSLSPGK

SEQ ID NO: 70 - DNA, 1545 bp, Artificial Sequence
  Synthetic
atggagttcggcctgagctggctgttcctggtggccatccttaagggcgtgcagtgcgccgtgacgttggacgagtccgggggcggcctccagacgcccgggggagcgctcagcctcgtctgcaaggcctccgggttcaccttcagcagtaacgccatgggttgggtgcgacaggcgcccggcaaggggctggagtgggtcgctggtattgatgatgatggtagtggcacaagatacgcgccggcggtgaagggccgtgccaccatctcgagggacaacgggcagagcacactgaggctgcagctgaacaacctcagggctgaggacaccggcacctactactgcgccaaagccgctggtggtagtggtctcgaggtgacatgtgaacccggtacgacgtttaaggataagtgcaacacatgtaggtgcggtagcgacggcaaatcagcgttctgtacccggaaattgtgctaccaggccgctggtggtagtggtggtagtggtgcttatatcgacgcatggggccacgggaccgaagtcatcgtctcctccgctagcaccaagggcccatcggtcttccccctggcaccctcctccaagagcacctctgggggcacagcggccctgggctgcctggtcaaggactacttccccgaaccggtgacggtgtcgtggaactcaggcgccctgaccagcggcgtgcacaccttcccggctgtcctacagtcctcaggactctactccctcagcagcgtggtgaccgtgccctccagcagcttgggcacccagacctacatctgcaacgtgaatcacaagcccagcaacaccaaggtggacaagaaagttgagcccaaatcttgtgacaaaactcacacatgcccaccgtgcccagcacctgaactcctggggggaccgtcagtcttcctcttccccccaaaacccaaggacaccctcatgatctcccggacccctgaggtcacatgcgtggtggtggacgtgagccacgaagaccctgaggtcaagttcaactggtacgtggacggcgtggaggtgcataatgccaagacaaagccgcgggaggagcagtacaacagcacgtaccgtgtggtcagcgtcctcaccgtcctgcaccaggactggctgaatggcaaggagtacaagtgcaaggtctccaacaaagccctcccagcccccatcgagaaaaccatctccaaagccaaagggcagccccgagaaccacaggtgtacaccctgcccccatcccgggatgagctgaccaagaaccaggtcagcctgacctgcctggtcaaaggcttctatcccagcgacatcgccgtggagtgggagagcaatgggcagccggagaacaactacaagaccacgcctcccgtgctggactccgacggctccttcttcctctacagcaagctcaccgtggacaagagcaggtggcagcaggggaacgtcttctcatgctccgtgatgcatgaggctctgcacaaccactacacacagaagagcctctccctgtctccgggtaaatga

SEQ ID NO: 71 - protein, 495 aa, Artificial Sequence
  Synthetic
AVTLDESGGGLQTPGGALSLVCKASGFTFSSNAMGWVRQAPGKGLEWVAGIDDDGSGTRYAPAVKGRATISRDNGQSTLRLQLNNLRAEDTGTYYCAKAAGGSGLEVTCEPGTTFKDKCNTCRCGSDGKSAFCTRKLCYQAAGGSGGSGAYIDAWGHGTEVIVSSASTKGPSVFPLAPSSKSTSGGTAALGCLVKDYFPEPVTVSWNSGALTSGVHTFPAVLQSSGLYSLSSVVTVPSSSLGTQTYICNVNHKPSNTKVDKKVEPKSCDKTHTCPPCPAPELLGGPSVFLFPPKPKDTLMISRTPEVTCVVVDVSHEDPEVKFNWYVDGVEVHNAKTKPREEQYNSTYRVVSVLTVLHQDWLNGKEYKCKVSNKALPAPIEKTISKAKGQPREPQVYTLPPSRDELTKNQVSLTCLVKGFYPSDIAVEWESNGQPENNYKTTPPVLDSDGSFFLYSKLTVDKSRWQQGNVFSCSVMHEALHNHYTQKSLSLSPGK

SEQ ID NO: 72 - DNA, 1557 bp, Artificial Sequence
  Synthetic
atggagttcggcctgagctggctgttcctggtggccatccttaagggcgtgcagtgcgccgtgacgttggacgagtccgggggcggcctccagacgcccgggggagcgctcagcctcgtctgcaaggcctccgggttcaccttcagcagtaacgccatgggttgggtgcgacaggcgcccggcaaggggctggagtgggtcgctggtattgatgatgatggtagtggcacaagatacgcgccggcggtgaagggccgtgccaccatctcgagggacaacgggcagagcacactgaggctgcagctgaacaacctcagggctgaggacaccggcacctactactgcgccaaagccgctggtggtagtggtggtagtggtgctctcgaggtgacatgtgaacccggtacgacgtttaaggataagtgcaacacatgtaggtgcggtagcgacggcaaatcagcgttctgtacccggaaattgtgctaccaggccgctggtggtagtggtggtagtggtgcttatatcgacgcatggggccacgggaccgaagtcatcgtctcctccgctagcaccaagggcccatcggtcttccccctggcaccctcctccaagagcacctctgggggcacagcggccctgggctgcctggtcaaggactacttccccgaaccggtgacggtgtcgtggaactcaggcgccctgaccagcggcgtgcacaccttcccggctgtcctacagtcctcaggactctactccctcagcagcgtggtgaccgtgccctccagcagcttgggcacccagacctacatctgcaacgtgaatcacaagcccagcaacaccaaggtggacaagaaagttgagcccaaatcttgtgacaaaactcacacatgcccaccgtgcccagcacctgaactcctggggggaccgtcagtcttcctcttccccccaaaacccaaggacaccctcatgatctcccggacccctgaggtcacatgcgtggtggtggacgtgagccacgaagaccctgaggtcaagttcaactggtacgtggacggcgtggaggtgcataatgccaagacaaagccgcgggaggagcagtacaacagcacgtaccgtgtggtcagcgtcctcaccgtcctgcaccaggactggctgaatggcaaggagtacaagtgcaaggtctccaacaaagccctcccagcccccatcgagaaaaccatctccaaagccaaagggcagccccgagaaccacaggtgtacaccctgcccccatcccgggatgagctgaccaagaaccaggtcagcctgacctgcctggtcaaaggcttctatcccagcgacatcgccgtggagtgggagagcaatgggcagccggagaacaactacaagaccacgcctcccgtgctggactccgacggctccttcttcctctacagcaagctcaccgtggacaagagcaggtggcagcaggggaacgtcttctcatgctccgtgatgcatgaggctctgcacaaccactacacacagaagagcctctccctgtctccgggtaaatga

SEQ ID NO: 73 - protein, 499 aa, Artificial Sequence
  Synthetic
AVTLDESGGGLQTPGGALSLVCKASGFTFSSNAMGWVRQAPGKGLEWVAGIDDDGSGTRYAPAVKGRATISRDNGQSTLRLQLNNLRAEDTGTYYCAKAAGGSGGSGALEVTCEPGTTFKDKCNTCRCGSDGKSAFCTRKLCYQAAGGSGGSGAYIDAWGHGTEVIVSSASTKGPSVFPLAPSSKSTSGGTAALGCLVKDYFPEPVTVSWNSGALTSGVHTFPAVLQSSGLYSLSSVVTVPSSSLGTQTYICNVNHKPSNTKVDKKVEPKSCDKTHTCPPCPAPELLGGPSVFLFPPKPKDTLMISRTPEVTCVVVDVSHEDPEVKFNWYVDGVEVHNAKTKPREEQYNSTYRVVSVLTVLHQDWLNGKEYKCKVSNKALPAPIEKTISKAKGQPREPQVYTLPPSRDELTKNQVSLTCLVKGFYPSDIAVEWESNGQPENNYKTTPPVLDSDGSFFLYSKLTVDKSRWQQGNVFSCSVMHEALHNHYTQKSLSLSPGK

SEQ ID NO: 74 - DNA, 795 bp, Artificial Sequence
  Synthetic
atggcctggattcctctacttctccccctcctcactctctgcacaggatccgaagccgcgctgactcagcctgcctcggtgtcagcaaacccaggagaaaccgtcaagatcacctgctccgggggtggcagcttggaagtgacgtgtgagcccggaacgacattcaaagacaagtgcaatacttgtcggtgcggttcagatgggaaatcggcggtctgcacaaagctctggtgtaaccagtactattatggctggtaccagcagaaggcacctggcagtgcccctgtcactctgatctattacaacaacaagagaccctcggacatcccttcacgattctccggttccctatccggctccacaaacacattaaccatcactggggtccgagccgatgacgaggctgtctatttctgtgggagtgcagacaacagtggtgctgcatttggggccgggacaaccctgacagtacttggtcagcccaaggctgccccttcggtcaccctgttcccgccctcctctgaggagcttcaagccaacaaggccacactggtgtgtctcataagtgacttctacccgggagccgtgacagtggcctggaaggcagatagcagccccgtcaaggcgggagtggagaccaccacaccctccaaacaaagcaacaacaagtacgcggccagcagctatctgagcctgacgcctgagcagtggaagtcccacagaagctacagctgccaggtcacgcatgaagggagcaccgtggagaagacagtggcccctacagaatgttcatag

SEQ ID NO: 75 - protein, 245 aa, Artificial Sequence
  Synthetic
ALTQPASVSANPGETVKITCSGGGSLEVTCEPGTTFKDKCNTCRCGSDGKSAVCTKLWCNQYYYGWYQQKAPGSAPVTLIYYNNKRPSDIPSRFSGSLSGSTNTLTITGVRADDEAVYFCGSADNSGAAFGAGTTLTVLGQPKAAPSVTLFPPSSEELQANKATLVCLISDFYPGAVTVAWKADSSPVKAGVETTTPSKQSNNKYAASSYLSLTPEQWKSHRSYSCQVTHEGSTVEKTVAPTECS

SEQ ID NO: 76 - DNA, 786 bp, Artificial Sequence
  Synthetic
atggcctggattcctctacttctccccctcctcactctctgcacaggatccgaagccgcgctgactcagcctgcctcggtgtcagcaaacccaggagaaaccgtcaagatcacctgctccgggggtggcagcacgtgtgagcccggaacgacattcaaagacaagtgcaatacttgtcggtgcggttcagatgggaaatcggcggtctgcacaaagctctggtgtaaccagtactattatggctggtaccagcagaaggcacctggcagtgcccctgtcactctgatctattacaacaacaagagaccctcggacatcccttcacgattctccggttccctatccggctccacaaacacattaaccatcactggggtccgagccgatgacgaggctgtctatttctgtgggagtgcagacaacagtggtgctgcatttggggccgggacaaccctgacagtacttggtcagcccaaggctgccccttcggtcaccctgttcccgccctcctctgaggagcttcaagccaacaaggccacactggtgtgtctcataagtgacttctacccgggagccgtgacagtggcctggaaggcagatagcagccccgtcaaggcgggagtggagaccaccacaccctccaaacaaagcaacaacaagtacgcggccagcagctatctgagcctgacgcctgagcagtggaagtcccacagaagctacagctgccaggtcacgcatgaagggagcaccgtggagaagacagtggcccctacagaatgttcatag

SEQ ID NO: 77 - protein, 242 aa, Artificial Sequence
  Synthetic
ALTQPASVSANPGETVKITCSGGGSTCEPGTTFKDKCNTCRCGSDGKSAVCTKLWCNQYYYGWYQQKAPGSAPVTLIYYNNKRPSDIPSRFSGSLSGSTNTLTITGVRADDEAVYFCGSADNSGAAFGAGTTLTVLGQPKAAPSVTLFPPSSEELQANKATLVCLISDFYPGAVTVAWKADSSPVKAGVETTTPSKQSNNKYAASSYLSLTPEQWKSHRSYSCQVTHEGSTVEKTVAPTECS

SEQ ID NO: 78 - DNA, 747 bp, Artificial Sequence
  Synthetic
atggcctggattcctctacttctccccctcctcactctctgcacaggatccgaagccgcgctgactcagcctgcctcggtgtcagcaaacccaggagaaaccgtcaagatcacctgctccgggggtggcagcacttgtcggtgcggttcagatgggaaatcggcggtctgcacaaagctctggtgtaaccagtactattatggctggtaccagcagaaggcacctggcagtgcccctgtcactctgatctattacaacaacaagagaccctcggacatcccttcacgattctccggttccctatccggctccacaaacacattaaccatcactggggtccgagccgatgacgaggctgtctatttctgtgggagtgcagacaacagtggtgctgcatttggggccgggacaaccctgacagtacttggtcagcccaaggctgccccttcggtcaccctgttcccgccctcctctgaggagcttcaagccaacaaggccacactggtgtgtctcataagtgacttctacccgggagccgtgacagtggcctggaaggcagatagcagccccgtcaaggcgggagtggagaccaccacaccctccaaacaaagcaacaacaagtacgcggccagcagctatctgagcctgacgcctgagcagtggaagtcccacagaagctacagctgccaggtcacgcatgaagggagcaccgtggagaagacagtggcccctacagaatgttcatag

SEQ ID NO: 79 - protein, 229 aa, Artificial Sequence
  Synthetic
ALTQPASVSANPGETVKITCSGGGSTCRCGSDGKSAVCTKLWCNQYYYGWYQQKAPGSAPVTLIYYNNKRPSDIPSRFSGSLSGSTNTLTITGVRADDEAVYFCGSADNSGAAFGAGTTLTVLGQPKAAPSVTLFPPSSEELQANKATLVCLISDFYPGAVTVAWKADSSPVKAGVETTTPSKQSNNKYAASSYLSLTPEQWKSHRSYSCQVTHEGSTVEKTVAPTECS

SEQ ID NO: 80 - DNA, 795 bp, Artificial Sequence
  Synthetic
atggcctggattcctctacttctccccctcctcactctctgcacaggatccgaagccgcgctgactcagcctgcctcggtgtcagcaaacccaggagaaaccgtcaagatcacctgctccgggggtggcagcctcgaggtgacatgtgaacccggtacgacgtttaaggataagtgcaacacatgtaggtgcggtagcgacggcaaatcagcgttctgtacccggaaattgtgctaccagtactattatggctggtaccagcagaaggcacctggcagtgcccctgtcactctgatctattacaacaacaagagaccctcggacatcccttcacgattctccggttccctatccggctccacaaacacattaaccatcactggggtccgagccgatgacgaggctgtctatttctgtgggagtgcagacaacagtggtgctgcatttggggccgggacaaccctgacagtacttggtcagcccaaggctgccccttcggtcaccctgttcccgccctcctctgaggagcttcaagccaacaaggccacactggtgtgtctcataagtgacttctacccgggagccgtgacagtggcctggaaggcagatagcagccccgtcaaggcgggagtggagaccaccacaccctccaaacaaagcaacaacaagtacgcggccagcagctatctgagcctgacgcctgagcagtggaagtcccacagaagctacagctgccaggtcacgcatgaagggagcaccgtggagaagacagtggcccctacagaatgttcatag

SEQ ID NO: 81 - protein, 245 aa, Artificial Sequence
  Synthetic
ALTQPASVSANPGETVKITCSGGGSLEVTCEPGTTFKDKCNTCRCGSDGKSAFCTRKLCYQYYYGWYQQKAPGSAPVTLIYYNNKRPSDIPSRFSGSLSGSTNTLTITGVRADDEAVYFCGSADNSGAAFGAGTTLTVLGQPKAAPSVTLFPPSSEELQANKATLVCLISDFYPGAVTVAWKADSSPVKAGVETTTPSKQSNNKYAASSYLSLTPEQWKSHRSYSCQVTHEGSTVEKTVAPTECS

SEQ ID NO: 82 - DNA, 786 bp, Artificial Sequence
  Synthetic
atggcctggattcctctacttctccccctcctcactctctgcacaggatccgaagccgcgctgactcagcctgcctcggtgtcagcaaacccaggagaaaccgtcaagatcacctgctccgggggtggcagcacatgtgaacccggtacgacgtttaaggataagtgcaacacatgtaggtgcggtagcgacggcaaatcagcgttctgtacccggaaattgtgctaccagtactattatggctggtaccagcagaaggcacctggcagtgcccctgtcactctgatctattacaacaacaagagaccctcggacatcccttcacgattctccggttccctatccggctccacaaacacattaaccatcactggggtccgagccgatgacgaggctgtctatttctgtgggagtgcagacaacagtggtgctgcatttggggccgggacaaccctgacagtacttggtcagcccaaggctgccccttcggtcaccctgttcccgccctcctctgaggagcttcaagccaacaaggccacactggtgtgtctcataagtgacttctacccgggagccgtgacagtggcctggaaggcagatagcagccccgtcaaggcgggagtggagaccaccacaccctccaaacaaagcaacaacaagtacgcggccagcagctatctgagcctgacgcctgagcagtggaagtcccacagaagctacagctgccaggtcacgcatgaagggagcaccgtggagaagacagtggcccctacagaatgttcatag

SEQ ID NO: 83 - protein, 242 aa, Artificial Sequence
  Synthetic
ALTQPASVSANPGETVKITCSGGGSTCEPGTTFKDKCNTCRCGSDGKSAFCTRKLCYQYYYGWYQQKAPGSAPVTLIYYNNKRPSDIPSRFSGSLSGSTNTLTITGVRADDEAVYFCGSADNSGAAFGAGTTLTVLGQPKAAPSVTLFPPSSEELQANKATLVCLISDFYPGAVTVAWKADSSPVKAGVETTTPSKQSNNKYAASSYLSLTPEQWKSHRSYSCQVTHEGSTVEKTVAPTECS

SEQ ID NO: 84 - DNA, 747 bp, Artificial Sequence
  Synthetic
atggcctggattcctctacttctccccctcctcactctctgcacaggatccgaagccgcgctgactcagcctgcctcggtgtcagcaaacccaggagaaaccgtcaagatcacctgctccgggggtggcagcacatgtaggtgcggtagcgacggcaaatcagcgttctgtacccggaaattgtgctaccagtactattatggctggtaccagcagaaggcacctggcagtgcccctgtcactctgatctattacaacaacaagagaccctcggacatcccttcacgattctccggttccctatccggctccacaaacacattaaccatcactggggtccgagccgatgacgaggctgtctatttctgtgggagtgcagacaacagtggtgctgcatttggggccgggacaaccctgacagtacttggtcagcccaaggctgccccttcggtcaccctgttcccgccctcctctgaggagcttcaagccaacaaggccacactggtgtgtctcataagtgacttctacccgggagccgtgacagtggcctggaaggcagatagcagccccgtcaaggcgggagtggagaccaccacaccctccaaacaaagcaacaacaagtacgcggccagcagctatctgagcctgacgcctgagcagtggaagtcccacagaagctacagctgccaggtcacgcatgaagggagcaccgtggagaagacagtggcccctacagaatgttcatag

SEQ ID NO: 85 - protein, 229 aa, Artificial Sequence
  Synthetic
ALTQPASVSANPGETVKITCSGGGSTCRCGSDGKSAFCTRKLCYQYYYGWYQQKAPGSAPVTLIYYNNKRPSDIPSRFSGSLSGSTNTLTITGVRADDEAVYFCGSADNSGAAFGAGTTLTVLGQPKAAPSVTLFPPSSEELQANKATLVCLISDFYPGAVTVAWKADSSPVKAGVETTTPSKQSNNKYAASSYLSLTPEQWKSHRSYSCQVTHEGSTVEKTVAPTECS

SEQ ID NO: 86 - protein, 125 aa, Artificial Sequence
  Synthetic
AVTLDESGGGLQTPGGALSLVCKASGFTFSSNAMGWVRQAPGKGLEWVAGIDDDGSGTRYAPAVKGRATISRDNGQSTLRLQLNNLRAEDTGIYYCTKCAYSSGCDYEGGYIDAWGHGTEVIVSS

SEQ ID NO: 87 - protein, 107 aa, Artificial Sequence
  Synthetic
ALTQPASVSANPGETVKITCSGGGSYAGSYYYGWYQQKAPGSAPVTLIYYNNKRPSDIPSRFSGSLSGSTNTLTITGVRADDEAVYFCGSADNSGAAFGAGTTLTVL

SEQ ID NO: 88 - DNA, 1563 bp, Artificial Sequence
  Synthetic
atggagttcggcctgagctggctgttcctggtggccatccttaagggcgtgcagtgcctcgaggtgacatgtgaacccggtacgacgtttaaggataagtgcaacacatgtaggtgcggtagcgacggcaaatcagcgttctgtacccggaaattgtgctaccagggaactggaggagggtcggggtcctcgtcagccgtgacgttggacgagtccgggggcggcctccagacgcccgggggagcgctcagcctcgtctgcaaggcctccgggttcaccttcagcagtaacgccatgggttgggtgcgacaggcgcccggcaaggggctggagtgggtcgctggtattgatgatgatggtagtggcacaagatacgcgccggcggtgaagggccgtgccaccatctcgagggacaacgggcagagcacactgaggctgcagctgaacaacctcagggctgaggacaccggcatctactactgcacgaaatgtgcttacagtagtggttgtgattatgaaggtggttatatcgacgcatggggccacgggaccgaagtcatcgtctcctccgctagcaccaagggcccatcggtcttccccctggcaccctcctccaagagcacctctgggggcacagcggccctgggctgcctggtcaaggactacttccccgaaccggtgacggtgtcgtggaactcaggcgccctgaccagcggcgtgcacaccttcccggctgtcctacagtcctcaggactctactccctcagcagcgtggtgaccgtgccctccagcagcttgggcacccagacctacatctgcaacgtgaatcacaagcccagcaacaccaaggtggacaagaaagttgagcccaaatcttgtgacaaaactcacacatgcccaccgtgcccagcacctgaactcctggggggaccgtcagtcttcctcttccccccaaaacccaaggacaccctcatgatctcccggacccctgaggtcacatgcgtggtggtggacgtgagccacgaagaccctgaggtcaagttcaactggtacgtggacggcgtggaggtgcataatgccaagacaaagccgcgggaggagcagtacaacagcacgtaccgtgtggtcagcgtcctcaccgtcctgcaccaggactggctgaatggcaaggagtacaagtgcaaggtctccaacaaagccctcccagcccccatcgagaaaaccatctccaaagccaaagggcagccccgagaaccacaggtgtacaccctgcccccatcccgggatgagctgaccaagaaccaggtcagcctgacctgcctggtcaaaggcttctatcccagcgacatcgccgtggagtgggagagcaatgggcagccggagaacaactacaagaccacgcctcccgtgctggactccgacggctccttcttcctctacagcaagctcaccgtggacaagagcaggtggcagcaggggaacgtcttctcatgctccgtgatgcatgaggctctgcacaaccactacacacagaagagcctctccctgtctccgggtaaatga

SEQ ID NO: 89 - protein, 501 aa, Artificial Sequence
  Synthetic
LEVTCEPGTTFKDKCNTCRCGSDGKSAFCTRKLCYQGTGGGSGSSSAVTLDESGGGLQTPGGALSLVCKASGFTFSSNAMGWVRQAPGKGLEWVAGIDDDGSGTRYAPAVKGRATISRDNGQSTLRLQLNNLRAEDTGIYYCTKCAYSSGCDYEGGYIDAWGHGTEVIVSSASTKGPSVFPLAPSSKSTSGGTAALGCLVKDYFPEPVTVSWNSGALTSGVHTFPAVLQSSGLYSLSSVVTVPSSSLGTQTYICNVNHKPSNTKVDKKVEPKSCDKTHTCPPCPAPELLGGPSVFLFPPKPKDTLMISRTPEVTCVVVDVSHEDPEVKFNWYVDGVEVHNAKTKPREEQYNSTYRVVSVLTVLHQDWLNGKEYKCKVSNKALPAPIEKTISKAKGQPREPQVYTLPPSRDELTKNQVSLTCLVKGFYPSDIAVEWESNGQPENNYKTTPPVLDSDGSFFLYSKLTVDKSRWQQGNVFSCSVMHEALHNHYTQKSLSLSPGK

SEQ ID NO: 90 - DNA, 1563 bp, Artificial Sequence
  Synthetic
atggagttcggcctgagctggctgttcctggtggccatccttaagggcgtgcagtgcttggaagtgacgtgtgagcccggaacgacattcaaagacaagtgcaatacttgtcggtgcggttcagatgggaaatcggcggtctgcacaaagctctggtgtaaccagggcaccggtggagggtcgggatccagctcagccgtgacgttggacgagtccgggggcggcctccagacgcccgggggagcgctcagcctcgtctgcaaggcctccgggttcaccttcagcagtaacgccatgggttgggtgcgacaggcgcccggcaaggggctggagtgggtcgctggtattgatgatgatggtagtggcacaagatacgcgccggcggtgaagggccgtgccaccatctcgagggacaacgggcagagcacactgaggctgcagctgaacaacctcagggctgaggacaccggcatctactactgcacgaaatgtgcttacagtagtggttgtgattatgaaggtggttatatcgacgcatggggccacgggaccgaagtcatcgtctcctccgctagcaccaagggcccatcggtcttccccctggcaccctcctccaagagcacctctgggggcacagcggccctgggctgcctggtcaaggactacttccccgaaccggtgacggtgtcgtggaactcaggcgccctgaccagcggcgtgcacaccttcccggctgtcctacagtcctcaggactctactccctcagcagcgtggtgaccgtgccctccagcagcttgggcacccagacctacatctgcaacgtgaatcacaagcccagcaacaccaaggtggacaagaaagttgagcccaaatcttgtgacaaaactcacacatgcccaccgtgcccagcacctgaactcctggggggaccgtcagtcttcctcttccccccaaaacccaaggacaccctcatgatctcccggacccctgaggtcacatgcgtggtggtggacgtgagccacgaagaccctgaggtcaagttcaactggtacgtggacggcgtggaggtgcataatgccaagacaaagccgcgggaggagcagtacaacagcacgtaccgtgtggtcagcgtcctcaccgtcctgcaccaggactggctgaatggcaaggagtacaagtgcaaggtctccaacaaagccctcccagcccccatcgagaaaaccatctccaaagccaaagggcagccccgagaaccacaggtgtacaccctgcccccatcccgggatgagctgaccaagaaccaggtcagcctgacctgcctggtcaaaggcttctatcccagcgacatcgccgtggagtgggagagcaatgggcagccggagaacaactacaagaccacgcctcccgtgctggactccgacggctccttcttcctctacagcaagctcaccgtggacaagagcaggtggcagcaggggaacgtcttctcatgctccgtgatgcatgaggctctgcacaaccactacacacagaagagcctctccctgtctccgggtaaatga

SEQ ID NO: 91 - protein, 501 aa, Artificial Sequence [sequence omitted]

SEQ ID NO: 92 - DNA, 1563 bp, Artificial Sequence
  Synthetic
atggagttcggcctgagctggctgttcctggtggccatccttaagggcgtgcagtgcgccgtgacgttggacgagtccgggggcggcctccagacgcccgggggagcgctcagcctcgtctgcaaggcctccgggttcaccttcagcagtaacgccatgggttgggtgcgacaggcgcccggcaaggggctggagtgggtcgctggtattgatgatgatggtagtggcacaagatacgcgccggcggtgaagggccgtgccaccatctcgagggacaacgggcagagcacactgaggctgcagctgaacaacctcagggctgaggacaccggcatctactactgcacgaaatgtgcttacagtagtggttgtgattatgaaggtggttatatcgacgcatggggccacgggaccgaagtcatcgtctcctccgctagcaccaagggcccatcggtcttccccctggcaccctcctccaagagcacctctgggggcacagcggccctgggctgcctggtcaaggactacttccccgaaccggtgacggtgtcgtggaactcaggcgccctgaccagcggcgtgcacaccttcccggctgtcctacagtcctcaggactctactccctcagcagcgtggtgaccgtgccctccagcagcttgggcacccagacctacatctgcaacgtgaatcacaagcccagcaacaccaaggtggacaagaaagttgagcccaaatcttgtgacaaaactcacacatgcccaccgtgcccagcacctgaactcctggggggaccgtcagtcttcctcttccccccaaaacccaaggacaccctcatgatctcccggacccctgaggtcacatgcgtggtggtggacgtgagccacgaagaccctgaggtcaagttcaactggtacgtggacggcgtggaggtgcataatgccaagacaaagccgcgggaggagcagtacaacagcacgtaccgtgtggtcagcgtcctcaccgtcctgcaccaggactggctgaatggcaaggagtacaagtgcaaggtctccaacaaagccctcccagcccccatcgagaaaaccatctccaaagccaaagggcagccccgagaaccacaggtgtacaccctgcccccatcccgggatgagctgaccaagaaccaggtcagcctgacctgcctggtcaaaggcttctatcccagcgacatcgccgtggagtgggagagcaatgggcagccggagaacaactacaagaccacgcctcccgtgctggactccgacggctccttcttcctctacagcaagctcaccgtggacaagagcaggtggcagcaggggaacgtcttctcatgctccgtgatgcatgaggctctgcacaaccactacacacagaagagcctctccctgtctccgggtaaagccgctggtggtagtggtctcgaggtgacatgtgaacccggtacgacgtttaaggataagtgcaacacatgtaggtgcggtagcgacggcaaatcagcgttctgtacccggaaattgtgctaccagggtagtggtgcttga

SEQ ID NO: 93 - protein, 501 aa, Artificial Sequence
  Synthetic
AVTLDESGGGLQTPGGALSLVCKASGFTFSSNAMGWVRQAPGKGLEWVAGIDDDGSGTRYAPAVKGRATISRDNGQSTLRLQLNNLRAEDTGIYYCTKCAYSSGCDYEGGYIDAWGHGTEVIVSSASTKGPSVFPLAPSSKSTSGGTAALGCLVKDYFPEPVTVSWNSGALTSGVHTFPAVLQSSGLYSLSSVVTVPSSSLGTQTYICNVNHKPSNTKVDKKVEPKSCDKTHTCPPCPAPELLGGPSVFLFPPKPKDTLMISRTPEVTCVVVDVSHEDPEVKFNWYVDGVEVHNAKTKPREEQYNSTYRVVSVLTVLHQDWLNGKEYKCKVSNKALPAPIEKTISKAKGQPREPQVYTLPPSRDELTKNQVSLTCLVKGFYPSDIAVEWESNGQPENNYKTTPPVLDSDGSFFLYSKLTVDKSRWQQGNVFSCSVMHEALHNHYTQKSLSLSPGKAAGGSGLEVTCEPGTTFKDKCNTCRCGSDGKSAFCTRKLCYQGSGA

SEQ ID NO: 94 - DNA, 1563 bp, Artificial Sequence
  Synthetic
atggagttcggcctgagctggctgttcctggtggccatccttaagggcgtgcagtgcgccgtgacgttggacgagtccgggggcggcctccagacgcccgggggagcgctcagcctcgtctgcaaggcctccgggttcaccttcagcagtaacgccatgggttgggtgcgacaggcgcccggcaaggggctggagtgggtcgctggtattgatgatgatggtagtggcacaagatacgcgccggcggtgaagggccgtgccaccatctcgagggacaacgggcagagcacactgaggctgcagctgaacaacctcagggctgaggacaccggcatctactactgcacgaaatgtgcttacagtagtggttgtgattatgaaggtggttatatcgacgcatggggccacgggaccgaagtcatcgtctcctccgctagcaccaagggcccatcggtcttccccctggcaccctcctccaagagcacctctgggggcacagcggccctgggctgcctggtcaaggactacttccccgaaccggtgacggtgtcgtggaactcaggcgccctgaccagcggcgtgcacaccttcccggctgtcctacagtcctcaggactctactccctcagcagcgtggtgaccgtgccctccagcagcttgggcacccagacctacatctgcaacgtgaatcacaagcccagcaacaccaaggtggacaagaaagttgagcccaaatcttgtgacaaaactcacacatgcccaccgtgcccagcacctgaactcctggggggaccgtcagtcttcctcttccccccaaaacccaaggacaccctcatgatctcccggacccctgaggtcacatgcgtggtggtggacgtgagccacgaagaccctgaggtcaagttcaactggtacgtggacggcgtggaggtgcataatgccaagacaaagccgcgggaggagcagtacaacagcacgtaccgtgtggtcagcgtcctcaccgtcctgcaccaggactggctgaatggcaaggagtacaagtgcaaggtctccaacaaagccctcccagcccccatcgagaaaaccatctccaaagccaaagggcagccccgagaaccacaggtgtacaccctgcccccatcccgggatgagctgaccaagaaccaggtcagcctgacctgcctggtcaaaggcttctatcccagcgacatcgccgtggagtgggagagcaatgggcagccggagaacaactacaagaccacgcctcccgtgctggactccgacggctccttcttcctctacagcaagctcaccgtggacaagagcaggtggcagcaggggaacgtcttctcatgctccgtgatgcatgaggctctgcacaaccactacacacagaagagcctctccctgtctccgggtaaagccgctggtggtagtggtttggaagtgacgtgtgagcccggaacgacattcaaagacaagtgcaatacttgtcggtgcggttcagatgggaaatcggcggtctgcacaaagctctggtgtaaccagggtagtggtgcttga

SEQ ID NO: 95 - protein, 501 aa, Artificial Sequence
  Synthetic
AVTLDESGGGLQTPGGALSLVCKASGFTFSSNAMGWVRQAPGKGLEWVAGIDDDGSGTRYAPAVKGRATISRDNGQSTLRLQLNNLRAEDTGIYYCTKCAYSSGCDYEGGYIDAWGHGTEVIVSSASTKGPSVFPLAPSSKSTSGGTAALGCLVKDYFPEPVTVSWNSGALTSGVHTFPAVLQSSGLYSLSSVVTVPSSSLGTQTYICNVNHKPSNTKVDKKVEPKSCDKTHTCPPCPAPELLGGPSVFLFPPKPKDTLMISRTPEVTCVVVDVSHEDPEVKFNWYVDGVEVHNAKTKPREEQYNSTYRVVSVLTVLHQDWLNGKEYKCKVSNKALPAPIEKTISKAKGQPREPQVYTLPPSRDELTKNQVSLTCLVKGFYPSDIAVEWESNGQPENNYKTTPPVLDSDGSFFLYSKLTVDKSRWQQGNVFSCSVMHEALHNHYTQKSLSLSPGKAAGGSGLEVTCEPGTTFKDKCNTCRCGSDGKSAVCTKLWCNQGSGA

SEQ ID NO: 96 - DNA, 837 bp, Artificial Sequence
  Synthetic
atggcctggattcctctacttctccccctcctcactctctgcacaggatccgaagccctcgaggtgacatgtgaacccggtacgacgtttaaggataagtgcaacacatgtaggtgcggtagcgacggcaaatcagcgttctgtacccggaaattgtgctaccagggaactggaggagggtcggggtcctcgtcagcgctgactcagcctgcctcggtgtcagcaaacccaggagaaaccgtcaagatcacctgctccgggggtggcagctatgctggaagttactattatggctggtaccagcagaaggcacctggcagtgcccctgtcactctgatctattacaacaacaagagaccctcggacatcccttcacgattctccggttccctatccggctccacaaacacattaaccatcactggggtccgagccgatgacgaggctgtctatttctgtgggagtgcagacaacagtggtgctgcatttggggccgggacaaccctgacagtacttggtcagcccaaggctgccccttcggtcaccctgttcccgccctcctctgaggagcttcaagccaacaaggccacactggtgtgtctcataagtgacttctacccgggagccgtgacagtggcctggaaggcagatagcagccccgtcaaggcgggagtggagaccaccacaccctccaaacaaagcaacaacaagtacgcggccagcagctatctgagcctgacgcctgagcagtggaagtcccacagaagctacagctgccaggtcacgcatgaagggagcaccgtggagaagacagtggcccctacagaatgttcatag

SEQ ID NO: 97 - protein, 259 aa, Artificial Sequence
  Synthetic
LEVTCEPGTTFKDKCNTCRCGSDGKSAFCTRKLCYQGTGGGSGSSSALTQPASVSANPGETVKITCSGGGSYAGSYYYGWYQQKAPGSAPVTLIYYNNKRPSDIPSRFSGSLSGSTNTLTITGVRADDEAVYFCGSADNSGAAFGAGTTLTVLGQPKAAPSVTLFPPSSEELQANKATLVCLISDFYPGAVTVAWKADSSPVKAGVETTTPSKQSNNKYAASSYLSLTPEQWKSHRSYSCQVTHEGSTVEKTVAPTECS

SEQ ID NO: 98 - DNA, 837 bp, Artificial Sequence
  Synthetic
atggcctggattcctctacttctccccctcctcactctctgcacaggatccgaagccttggaagtgacgtgtgagcccggaacgacattcaaagacaagtgcaatacttgtcggtgcggttcagatgggaaatcggcggtctgcacaaagctctggtgtaaccagggcaccggtggagggtcgggatccagctcagcgctgactcagcctgcctcggtgtcagcaaacccaggagaaaccgtcaagatcacctgctccgggggtggcagctatgctggaagttactattatggctggtaccagcagaaggcacctggcagtgcccctgtcactctgatctattacaacaacaagagaccctcggacatcccttcacgattctccggttccctatccggctccacaaacacattaaccatcactggggtccgagccgatgacgaggctgtctatttctgtgggagtgcagacaacagtggtgctgcatttggggccgggacaaccctgacagtacttggtcagcccaaggctgccccttcggtcaccctgttcccgccctcctctgaggagcttcaagccaacaaggccacactggtgtgtctcataagtgacttctacccgggagccgtgacagtggcctggaaggcagatagcagccccgtcaaggcgggagtggagaccaccacaccctccaaacaaagcaacaacaagtacgcggccagcagctatctgagcctgacgcctgagcagtggaagtcccacagaagctacagctgccaggtcacgcatgaagggagcaccgtggagaagacagtggcccctacagaatgttcatag

SEQ ID NO: 99 - protein, 259 aa, Artificial Sequence
  Synthetic
LEVTCEPGTTFKDKCNTCRCGSDGKSAVCTKLWCNQGTGGGSGSSSALTQPASVSANPGETVKITCSGGGSYAGSYYYGWYQQKAPGSAPVTLIYYNNKRPSDIPSRFSGSLSGSTNTLTITGVRADDEAVYFCGSADNSGAAFGAGTTLTVLGQPKAAPSVTLFPPSSEELQANKATLVCLISDFYPGAVTVAWKADSSPVKAGVETTTPSKQSNNKYAASSYLSLTPEQWKSHRSYSCQVTHEGSTVEKTVAPTECS

SEQ ID NO: 100 - DNA, 837 bp, Artificial Sequence
  Synthetic
atggcctggattcctctacttctccccctcctcactctctgcacaggatccgaagccgcgctgactcagcctgcctcggtgtcagcaaacccaggagaaaccgtcaagatcacctgctccgggggtggcagctatgctggaagttactattatggctggtaccagcagaaggcacctggcagtgcccctgtcactctgatctattacaacaacaagagaccctcggacatcccttcacgattctccggttccctatccggctccacaaacacattaaccatcactggggtccgagccgatgacgaggctgtctatttctgtgggagtgcagacaacagtggtgctgcatttggggccgggacaaccctgacagtacttggtcagcccaaggctgccccttcggtcaccctgttcccgccctcctctgaggagcttcaagccaacaaggccacactggtgtgtctcataagtgacttctacccgggagccgtgacagtggcctggaaggcagatagcagccccgtcaaggcgggagtggagaccaccacaccctccaaacaaagcaacaacaagtacgcggccagcagctatctgagcctgacgcctgagcagtggaagtcccacagaagctacagctgccaggtcacgcatgaagggagcaccgtggagaagacagtggcccctacagaatgttcagccgctggtggtagtggtctcgaggtgacatgtgaacccggtacgacgtttaaggataagtgcaacacatgtaggtgcggtagcgacggcaaatcagcgttctgtacccggaaattgtgctaccagggtagtggtgcttag

SEQ ID NO: 101 - protein, 259 aa, Artificial Sequence
  Synthetic
ALTQPASVSANPGETVKITCSGGGSYAGSYYYGWYQQKAPGSAPVTLIYYNNKRPSDIPSRFSGSLSGSTNTLTITGVRADDEAVYFCGSADNSGAAFGAGTTLTVLGQPKAAPSVTLFPPSSEELQANKATLVCLISDFYPGAVTVAWKADSSPVKAGVETTTPSKQSNNKYAASSYLSLTPEQWKSHRSYSCQVTHEGSTVEKTVAPTECSAAGGSGLEVTCEPGTTFKDKCNTCRCGSDGKSAFCTRKLCYQGSGA

SEQ ID NO: 102 - DNA, 837 bp, Artificial Sequence
  Synthetic
atggcctggattcctctacttctccccctcctcactctctgcacaggatccgaagccgcgctgactcagcctgcctcggtgtcagcaaacccaggagaaaccgtcaagatcacctgctccgggggtggcagctatgctggaagttactattatggctggtaccagcagaaggcacctggcagtgcccctgtcactctgatctattacaacaacaagagaccctcggacatcccttcacgattctccggttccctatccggctccacaaacacattaaccatcactggggtccgagccgatgacgaggctgtctatttctgtgggagtgcagacaacagtggtgctgcatttggggccgggacaaccctgacagtacttggtcagcccaaggctgccccttcggtcaccctgttcccgccctcctctgaggagcttcaagccaacaaggccacactggtgtgtctcataagtgacttctacccgggagccgtgacagtggcctggaaggcagatagcagccccgtcaaggcgggagtggagaccaccacaccctccaaacaaagcaacaacaagtacgcggccagcagctatctgagcctgacgcctgagcagtggaagtcccacagaagctacagctgccaggtcacgcatgaagggagcaccgtggagaagacagtggcccctacagaatgttcagccgctggtggtagtggtttggaagtgacgtgtgagcccggaacgacattcaaagacaagtgcaatacttgtcggtgcggttcagatgggaaatcggcggtctgcacaaagctctggtgtaaccagggtagtggtgcttag

SEQ ID NO: 103 - protein, 259 aa, Artificial Sequence
  Synthetic
ALTQPASVSANPGETVKITCSGGGSYAGSYYYGWYQQKAPGSAPVTLIYYNNKRPSDIPSRFSGSLSGSTNTLTITGVRADDEAVYFCGSADNSGAAFGAGTTLTVLGQPKAAPSVTLFPPSSEELQANKATLVCLISDFYPGAVTVAWKADSSPVKAGVETTTPSKQSNNKYAASSYLSLTPEQWKSHRSYSCQVTHEGSTVEKTVAPTECSAAGGSGLEVTCEPGTTFKDKCNTCRCGSDGKSAVCTKLWCNQGSGA

SEQ ID NO: 104 - protein, 259 aa, Artificial Sequence; identical to SEQ ID NO: 99
  Synthetic

SEQ ID NO: 105 - DNA, 837 bp, Artificial Sequence; identical to SEQ ID NO: 100
  Synthetic

SEQ ID NO: 106 - protein, 259 aa, Artificial Sequence; identical to SEQ ID NO: 101
  Synthetic

SEQ ID NO: 107 - DNA, 837 bp, Artificial Sequence; identical to SEQ ID NO: 102
  Synthetic

SEQ ID NO: 108 - protein, 259 aa, Artificial Sequence; identical to SEQ ID NO: 103
  Synthetic

SEQ ID NO: 109 - protein, 118 aa, artificial sequence
  Synthetic
QVTLKESGPVLVKPTETLTLTCTVSGFSLSRGKMGVSWIRQPPGKALEWLAHIFSSDEKSYRTSLKSRLTISKDTSKNQVVLTMTNMDPVDTATYYCARIRAGGIDYWGQGTLVTVSS

SEQ ID NO: 110 - DNA, 354 bp, artificial sequence
  Synthetic
caggtcaccttgaaggagtctggtcctgtgctggtgaaacccacagagaccctcacgctgacctgcaccgtctctgggttctcactcagcaggggtaaaatgggtgtgagctggatccgtcagcccccagggaaggccctggagtggcttgcacacattttttcgagtgacgaaaaatcctacaggacatcgctgaagagcaggctcaccatctccaaggacacctccaaaaaccaggtggtccttacaatgaccaacatggaccctgtggacacagccacgtattactgtgcacggatacgacgtggaggaattgactactggggccagggaaccctggtcactgtctcctca

SEQ ID NO: 111 - protein, 118 aa, artificial
  Synthetic
QVTLKESGPVLVKPTETLTLTCTVSGFSLSRGKMGVSWIRQPPGKALEWLAHIFSSDEKSYRTSLKSRLTISKDTSKNQVVLTMTNMDPVDTATYYCARIRRGGIDYWGQGTLVTVSS

SEQ ID NO: 112 - protein, 121 aa, artificial sequence
  Synthetic
QVQLQQSGPGLVKPSQTLSLTCAISGDSVSSTSAAWNWIRQSPSRGLEWLGRTYYRSKWYNDYAVSVKSRITINPDTSKNQFSLQLNSVTPEDTAVYYCARDPFGVPFDIWGQGTMVTVSS

SEQ ID NO: 113 - protein, 107 aa, artificial sequence
  Synthetic
QPVLTQPPSVSVSPGQTASITCSGDKLGDKFAYWYQQKPGHSPVLVIYQDNKRPSGIPGRFSGSNSGNTATLTISGTQAMDEADYYCQAWDSSTAVFGTGTKVTVLA

SEQ ID NO: 114 - DNA, 318 bp, artificial sequence
  Synthetic
  misc_feature (246)..(246): n is a, c, g, or t
cagccagtgctgactcagcccccctcactgtccgtgtccccaggacagacagccagcatcacctgctctggagagaaattgggggataaatatgcttactggtatcagcagaagccaggccagtcccctgtgttggtcatgtatcaagataaacagcggccctcagggatccctgagcgattctctggctccaactctgggaacacagccactctgaccatcagcgggacccaggctatggatgangctgactattactgtcaggcgtgggacagcagcactgcggtattcggcggagggaccaagctgaccgtccta

SEQ ID NO: 115 - protein, 106 aa, artificial sequence
  Synthetic
QPVLTQPPSLSVSPGQTASITCSGEKLGDKYAYWYQQKPGQSPVLVMYQDKQRPSGIPERFSGSNSGNTATLTISGTQAMDEADYYCQAWDSSTAVFGGGTKLTVL

SEQ ID NO: 116 - protein, 120 aa, artificial sequence
  Synthetic
SYVLTQPPSVSVAPGQTARITCGGNNIGSKNVHWYQQKPGQAPVLVVYDDSDRPSGIPERFSGSNSGNTATLTVSRVEAGDEADYYCQVWDTTTDHVVFGGGTKLTVLAAAGSEQKLISE

SEQ ID NO: 117 - DNA, 324 bp, artificial sequence
  Synthetic
tcctatgagctgatacagccaccctcggtgtcagtggccccaggacagacggccaccattacctgtgcgggagacaaccttgggaagaaacgtgtgcactggtaccagcagaggccaggccaggcccctgtgttggtcatctatgatgatagcgaccggccctcagggatccctgaccgattctctgcctccaactctgggaacacggccaccctgaccatcactaggggcgaagccggggatgaggccgactattattgtcaggtgtgggacattgctactgatcatgtggtcttcggcggagggaccaagctcaccgtccta

SEQ ID NO: 118 - protein, 120 aa, artificial sequence
  Synthetic
SYELIQPPSVSVAPGQTATITCAGDNLGKKRVHWYQQRPGQAPVLVIYDDSDRPSGIPDRFSASNSGNTATLTITRGEAGDEADYYCQVWDIATDHVVFGGGTKLTVLAAAGSEQKLISE

SEQ ID NO: 119 - protein, 5 aa, artificial sequence
  Synthetic
RGKMG

SEQ ID NO: 120 - protein, 5 aa, artificial sequence
  Synthetic
STSAA

SEQ ID NO: 121 - protein, 7 aa, artificial sequence
  Synthetic
GFSLSRG

SEQ ID NO: 122 - protein, 7 aa, artificial sequence
  Synthetic
GDSVSST

SEQ ID NO: 123 - protein, 16 aa, artificial sequence
  Synthetic
LAHIFSSDEKSYRTSL

SEQ ID NO: 124 - protein, 16 aa, artificial sequence
  Synthetic
LGRTYYRSKWYNDYAV

SEQ ID NO: 125 - protein, 5 aa, artificial sequence
  Synthetic
HIFSS

SEQ ID NO: 126 - protein, 5 aa, artificial sequence
  Synthetic
RTYYR

SEQ ID NO: 127 - protein, 8 aa, artificial sequence
  Synthetic
YYCARIRA

SEQ ID NO: 128 - protein, 8 aa, artificial sequence
  Synthetic
YYCARIRR

SEQ ID NO: 129 - protein, 8 aa, artificial sequence
  Synthetic
AVYYCARD

SEQ ID NO: 130 - protein, 7 aa, artificial sequence
  Synthetic
YYCARIR

SEQ ID NO: 131 - protein, 7 aa, artificial sequence
  Synthetic
AVYYCAR

SEQ ID NO: 132 - protein, 11 aa, artificial sequence
  Synthetic
GDKLGDKFAYW

SEQ ID NO: 133 - protein, 11 aa, artificial sequence
  Synthetic
GEKLGDKYAYW

SEQ ID NO: 134 - protein, 11 aa, artificial sequence
  Synthetic
GNNIGSKNVHW

SEQ ID NO: 135 - protein, 11 aa, artificial sequence
  Synthetic
GDNLGKKRVHW

SEQ ID NO: 136 - protein, 16 aa, artificial sequence
  Synthetic
AGDNLGKKRVHWYQQR

SEQ ID NO: 137 - protein, 7 aa, artificial sequence
  Synthetic
DNKRPSG

SEQ ID NO: 138 - protein, 7 aa, artificial sequence
  Synthetic
DKQRPSG

SEQ ID NO: 139 - protein, 11 aa, artificial sequence
  Synthetic
DKQRPSGIPER

SEQ ID NO: 140 - protein, 7 aa, artificial sequence
  Synthetic
DSDRPSG

SEQ ID NO: 141 - protein, 14 aa, artificial sequence
  Synthetic
DSDRPSGIPDRFSA

SEQ ID NO: 142 - protein, 9 aa, artificial sequence
  Synthetic
AWDSSTAVF

SEQ ID NO: 143 - protein, 16 aa, artificial sequence
  Synthetic
AWDSSTAVFGGGTKLT

SEQ ID NO: 144 - protein, 9 aa, artificial sequence
  Synthetic
VWDTTTDHV

SEQ ID NO: 145 - protein, 9 aa, artificial sequence
  Synthetic
VWDIATDHV

SEQ ID NO: 146 - protein, 29 aa, artificial sequence
  Synthetic
  misc_feature (8)..(8): Xaa can be any naturally occurring amino acid
  misc_feature (16)..(16): Xaa can be any naturally occurring amino acid
YYCARIRXWHEREINXATPSITINISARR

SEQ ID NO: 147 - protein, 53 aa, artificial sequence
  Synthetic
  misc_feature (2)..(2): Xaa can be any naturally occurring amino acid
  misc_feature (8)..(8): Xaa can be any naturally occurring amino acid
  misc_feature (19)..(19): Xaa can be any naturally occurring amino acid
  misc_feature (40)..(40): Xaa can be any naturally occurring amino acid
GXKLGDKXAYWWHEREINXATPSITINISDREWHEREINXATPSITINISFRY

SEQ ID NO: 148 - protein, 95 aa, artificial sequence
  Synthetic
  misc_feature (2)..(2): Xaa can be any naturally occurring amino acid
  misc_feature (4)..(4): Xaa can be any naturally occurring amino acid
  misc_feature (6)..(6): Xaa can be any naturally occurring amino acid
  misc_feature (8)..(8): Xaa can be any naturally occurring amino acid
  misc_feature (19)..(19): Xaa can be any naturally occurring amino acid
  misc_feature (40)..(40): Xaa can be any naturally occurring amino acid
  misc_feature (61)..(61): Xaa can be any naturally occurring amino acid
  misc_feature (82)..(82): Xaa can be any naturally occurring amino acid
GXNXGXKXVHWWHEREINXATPSITINISNRDWHEREINXATPSITINISIRLWHEREINXATPSITINISSRKWHEREINXATPSITINISNRR

SEQ ID NO: 149 - protein, 51 aa, artificial sequence
  Synthetic
  misc_feature (2)..(3): Xaa can be any naturally occurring amino acid
  misc_feature (15)..(15): Xaa can be any naturally occurring amino acid
  misc_feature (37)..(37): Xaa can be any naturally occurring amino acid
DXXRPSGWHEREINXATPSITINISNKRSWHEREINXATPSITINISKQRD

SEQ ID NO: 150 - protein, 51 aa, artificial sequence
  Synthetic
  misc_feature (4)..(5): Xaa can be any naturally occurring amino acid
  misc_feature (17)..(17): Xaa can be any naturally occurring amino acid
  misc_feature (38)..(38): Xaa can be any naturally occurring amino acid
VWDXXTDHVWHEREINXATPSITINISTRIWHEREINXATPSITINISTRA

SEQ ID NO: 151 - protein, 268 aa, artificial sequence
  Synthetic
QVTLKESGPVLVKPTETLTLTCTVSGFSLSRGKMGVSWIRQPPGKALEWLAHIFSSDEKSYRTSLKSRLTISKDTSKNQVVLTMTNMDPVDTATYYCARIRAGGIDYWGQGTLVTVSSKLSGSASAPKLEEGEFSEARVQPVLTQPPSVSVSPGQTASITCSGDKLGDKFAYWYQQKPGHSPVLVIYQDNKRPSGIPGRFSGSNSGNTATLTISGTQAMDEADYYCQAWDSSTAVFGTGTKVTVLAAAGSEQKLISEEDLNSHHHHHH

SEQ ID NO: 152 - protein, 271 aa, artificial sequence
  Synthetic
QVTLKESGPVLVKPTETLTLTCTVSGFSLSNARMGVSWIRQPPGKALEWLAHIFSNDEKSYSTSLKSRLTISKDTSKSQVVLTMTNMDPVDTATYYCARMAILTAGGMDVWGQGTTVTVSSKLSGSASAPKLEEGEFSEARVSYVLTQPPSVSASPGQTASITCSGDKLGDKYVSWYQQKPGRSPVLVIYRDTKRPSGIPERFSGSNYGNTATLTISGTQAVDEADYYCQAWDSGSGVFGGGTKVTVLAAAGSEQKLISEEDLNSHHHHHH

SEQ ID NO: 153 - protein, 272 aa, artificial sequence
  Synthetic
QITLKESGPVLVKPTETLTLTCTVSGFSLSNARMGVSWIRQPPGKALEWLAHIFSNDEKSYSTSLKSRLTISKDTSKSQVVLTMTNMDPVDTATYYCARMRYSSSLYGMDVWGQGTRVTVSSKLSGSASAPKLEEGEFSEARVSYELIQPPSVSVSPGQTASITCSGDKLGDKYVSWYQQKPGRSPVLVIYRDTKRPSGIPERFSGSNSGNTATLTISGTQAMDEADYYCQAWDSSTVVFGGGTKLTVLAAAGSEQKLISEEDLNSHHHHHH

SEQ ID NO: 154 - protein, 273 aa, artificial sequence
  Synthetic
EVQLQQSGPGLVKPSQTLSLTCAISGDSVSSKRAAWDWIRQSPSRGLEWLGRTYYRSKWFNDYAISVKSRITINADTSRNQFSLQLNSVTPEDTAVYYCVKSNSGTGAFDSWGQGTLVTVSSKLSGSASAPKLEEGEFSEARVQPGLTQPPSVSVSPGQTARITCSRDKLGDKYVSWYQQKPGQSPVVVMYKDNKRPSGIPERFSGSNSGNTATLTISGTQAMDEADYYCQAWDSSTAGVFGGGTKLTVLAAAGSEQKLISEEDLNSHHHHHH

SEQ ID NO: 155 - protein, 273 aa, artificial sequence
  Synthetic
QVQLQQSGPGLVKPSQTLSLTCAISGDSVSSTSAAWNWIRQSPSRGLEWLGRTYYRSKWYNDYAVSVKSRITINPDTSKNQFSLQLNSVTPEDTAVYYCARDPFGVPFDIWGQGTMVTVSSKLSGSASAPKLEEGEFSEARVSYVLTQPPSVSVAPGQTARITCGGNNIGSKNVHWYQQKPGQAPVLVVYDDSDRPSGIPERFSGSNSGNTATLTVSRVEAGDEADYYCQVWDTTTDHVVFGGGTKLTVLAAAGSEQKLISEEDLNSHHHHHH

SEQ ID NO: 156 - protein, 273 aa, artificial sequence
  Synthetic
QVQLQQSGPGLVKPSQTLSLTCAISGDSVSSNSAAWNWIRQSPSRGLEWLGRTYYRSKWYNDYAVSVKSRITINPDTSKNQFSLQLNSVTPEDTAVYYCARDPFGVPFDIWGQGTMVTVSSKLSGSASAPKLEEGEFSEARVSYVLTQPPSVSVAPGQTARVTCGGNNIRSKNVHWYQQKPGQAPVLVVYDDTDRPSGIPERFSGSNSGNTATLTVSRVEAGDEADYYCQVWDTTTDHVVFGGGTKLTVLAAAGSEQKLISEEDLNSHHHHHH

SEQ ID NO: 157 - protein, 273 aa, artificial sequence
  Synthetic
QVQLQQSGPGLVKPSQTLSLTCAISGDSVSSNSAAWNWIRQSPSRGLEWLGRTYYRSKWYNDYAVSVKSRITINPDTSKNQFSLQLNSVTPEDTAVYYCARDPFGVPFDIWGQGTMVTVSSKLSGSASAPKLEEGEFSEARVSYELTQLPSVSVAPGQTARVTCGGNNIRSKNVHWYQQKPGQAPVLVVYDDTDRPSGIPERFSGSNSGNTATLTVSRVEAGDEADYYCQVWDTTTDHVVFGGGTKVTVLAAAGSEQKLISEEDLNSHHHHHH

SEQ ID NO: 158 - DNA, 984 bp, homo sapiens
gcctccaccaagggcccatccgtcttccccctggcgccctgctccaggagcacctccgagagcacagccgccctgggctgcctggtcaaggactacttccccgaaccggtgacggtgtcgtggaactcaggcgccctgaccagcggcgtgcacaccttcccggctgtcctacagtcctcaggactctactccctcagcagcgtggtgaccgtgccctccagcagcttgggcacgaagacctacacctgcaacgtagatcacaagcccagcaacaccaaggtggacaagagagttgagtccaaatatggtcccccatgcccatcatgcccagcacctgagttcctggggggaccatcagtcttcctgttccccccaaaacccaaggacactctcatgatctcccggacccctgaggtcacgtgcgtggtggtggacgtgagccaggaagaccccgaggtccagttcaactggtacgtggatggcgtggaggtgcataatgccaagacaaagccgcgggaggagcagttcaacagcacgtaccgtgtggtcagcgtcctcaccgtcctgcaccaggactggctgaacggcaaggagtacaagtgcaaggtctccaacaaaggcctcccgtcctccatcgagaaaaccatctccaaagccaaagggcagccccgagagccacaggtgtacaccctgcccccatcccaggaggagatgaccaagaaccaggtcagcctgacctgcctggtcaaaggcttctaccccagcgacatcgccgtggagtgggagagcaatgggcagccggagaacaactacaagaccacgcctcccgtgctggactccgacggctccttcttcctctacagcaggctaaccgtggacaagagcaggtggcaggaggggaatgtcttctcatgctccgtgatgcatgaggctctgcacaaccactacacacagaagagcctctccctgtctctcgggaaatga

SEQ ID NO: 159 - protein, 327 aa, homo sapiens
ASTKGPSVFPLAPCSRSTSESTAALGCLVKDYFPEPVTVSWNSGALTSGVHTFPAVLQSSGLYSLSSVVTVPSSSLGTKTYTCNVDHKPSNTKVDKRVESKYGPPCPSCPAPEFLGGPSVFLFPPKPKDTLMISRTPEVTCVVVDVSQEDPEVQFNWYVDGVEVHNAKTKPREEQFNSTYRVVSVLTVLHQDWLNGKEYKCKVSNKGLPSSIEKTISKAKGQPREPQVYTLPPSQEEMTKNQVSLTCLVKGFYPSDIAVEWESNGQPENNYKTTPPVLDSDGSFFLYSRLTVDKSRWQEGNVFSCSVMHEALHNHYTQKSLSLSLGK

SEQ ID NO: 160 - DNA, 984 bp, artificial sequence
  Synthetic
gcctccaccaagggcccatccgtcttccccctggcgccctgctccaggagcacctccgagagcacagccgccctgggctgcctggtcaaggactacttccccgaaccggtgacggtgtcgtggaactcaggcgccctgaccagcggcgtgcacaccttcccggctgtcctacagtcctcaggactctactccctcagcagcgtggtgaccgtgccctccagcagcttgggcacgaagacctacacctgcaacgtagatcacaagcccagcaacaccaaggtggacaagagagttgagtccaaatatggtcccccatgcccaccatgcccagcacctgagttcctggggggaccatcagtcttcctgttccccccaaaacccaaggacactctcatgatctcccggacccctgaggtcacgtgcgtggtggtggacgtgagccaggaagaccccgaggtccagttcaactggtacgtggatggcgtggaggtgcataatgccaagacaaagccgcgggaggagcagttcaacagcacgtaccgtgtggtcagcgtcctcaccgtcctgcaccaggactggctgaacggcaaggagtacaagtgcaaggtctccaacaaaggcctcccgtcctccatcgagaaaaccatctccaaagccaaagggcagccccgagagccacaggtgtacaccctgcccccatcccaggaggagatgaccaagaaccaggtcagcctgacctgcctggtcaaaggcttctaccccagcgacatcgccgtggagtgggagagcaatgggcagccggagaacaactacaagaccacgcctcccgtgctggactccgacggctccttcttcctctacagcaggctaaccgtggacaagagcaggtggcaggaggggaatgtcttctcatgctccgtgatgcatgaggctctgcacaaccactacacacagaagagcctctccctgtctctcgggaaatga

SEQ ID NO: 161 - protein, 327 aa, artificial sequence
  Synthetic
ASTKGPSVFPLAPCSRSTSESTAALGCLVKDYFPEPVTVSWNSGALTSGVHTFPAVLQSSGLYSLSSVVTVPSSSLGTKTYTCNVDHKPSNTKVDKRVESKYGPPCPPCPAPEFLGGPSVFLFPPKPKDTLMISRTPEVTCVVVDVSQEDPEVQFNWYVDGVEVHNAKTKPREEQFNSTYRVVSVLTVLHQDWLNGKEYKCKVSNKGLPSSIEKTISKAKGQPREPQVYTLPPSQEEMTKNQVSLTCLVKGFYPSDIAVEWESNGQPENNYKTTPPVLDSDGSFFLYSRLTVDKSRWQEGNVFSCSVMHEALHNHYTQKSLSLSLGK

SEQ ID NO: 162 - DNA, 981 bp, homo sapiens
gcctccaccaagggcccatcggtcttccccctggcgccctgctccaggagcacctccgagagcacagcggccctgggctgcctggtcaaggactacttccccgaaccggtgacggtgtcgtggaactcaggcgctctgaccagcggcgtgcacaccttcccagctgtcctacagtcctcaggactctactccctcagcagcgtggtgaccgtgccctccagcaacttcggcacccagacctacacctgcaacgtagatcacaagcccagcaacaccaaggtggacaagacagttgagcgcaaatgttgtgtcgagtgcccaccgtgcccagcaccacctgtggcaggaccgtcagtcttcctcttccccccaaaacccaaggacaccctcatgatctcccggacccctgaggtcacgtgcgtggtggtggacgtgagccacgaagaccccgaggtccagttcaactggtacgtggacggcgtggaggtgcataatgccaagacaaagccacgggaggagcagttcaacagcacgttccgtgtggtcagcgtcctcaccgttgtgcaccaggactggctgaacggcaaggagtacaagtgcaaggtctccaacaaaggcctcccagcccccatcgagaaaaccatctccaaaaccaaagggcagccccgagaaccacaggtgtacaccctgcccccatcccgggaggagatgaccaagaaccaggtcagcctgacctgcctggtcaaaggcttctaccccagcgacatcgccgtagagtgggagagcaatgggcagccggagaacaactacaagaccacacctcccatgctggactccgacggctccttcttcctctacagcaagctcaccgtggacaagagcaggtggcagcaggggaacgtcttctcatgctccgtgatgcatgaggctctgcacaaccactacacgcagaagagcctctccctgtctcccgggaaatga

SEQ ID NO: 163 - protein, 326 aa, homo sapiens
ASTKGPSVFPLAPCSRSTSESTAALGCLVKDYFPEPVTVSWNSGALTSGVHTFPAVLQSSGLYSLSSVVTVPSSNFGTQTYTCNVDHKPSNTKVDKTVERKCCVECPPCPAPPVAGPSVFLFPPKPKDTLMISRTPEVTCVVVDVSHEDPEVQFNWYVDGVEVHNAKTKPREEQFNSTFRVVSVLTVVHQDWLNGKEYKCKVSNKGLPAPIEKTISKTKGQPREPQVYTLPPSREEMTKNQVSLTCLVKGFYPSDIAVEWESNGQPENNYKTTPPMLDSDGSFFLYSKLTVDKSRWQQGNVFSCSVMHEALHNHYTQKSLSLSPGK

SEQ ID NO: 164 - protein, 240 aa, rattus
MSFSNTLVFLLFLLKGILCEVQLVESGGGLVQPGRSLKLSCLVSGFTFSNFGMNWIRQAPGKGLEWVASISSGGTYIYHADTLKGRFTISRENAKNTLYLQMTSLRSEDTALYYCARGPYHSRYIPYLMDAWGQGASVTVSSAETTAPSVYPLAPGTALKSNSMVTLGCLVKGYFPEPVTVTWNSGALSSGVHTFPAVLQSGLYTLTSSVTVPSSTWPSQTVTCNVAHPASSTKVDKKIV

SEQ ID NO: 165 - protein, 240 aa, rattus
MGVPTQLLGLLLLWITDAICDIQMTQSPGSLCASLGETVTIECRASDDIYSNLAWYQQKPGNSPQLLIFDGNRLADGVPSRFSGSGSGTQYSLKMKSLQFEDVASYFCQQYNNYPLTFGSGTKLEIKRADAAPTVSIFPPSMEQLTSGGATVVCFVNNFYPRDISVKWKIDGSEQRDGVLDSVTDQDSKDSTYSMSSTLSLTKVEYERHNLYTCEVVHKTSSSPVVKSFNRNEKGEFQHT

SEQ ID NO: 166 - protein, 9 aa, rattus
GFTFSNFGM

SEQ ID NO: 167 - protein, 9 aa, rattus
SISSGGTYI

SEQ ID NO: 168 - protein, 14 aa, rattus
GPYHSRYIPYLMDA

SEQ ID NO: 169 - protein, 11 aa, rattus
RASDDIYSNLA

SEQ ID NO: 170 - protein, 7 aa, rattus
DGNRLAD

SEQ ID NO: 171 - protein, 9 aa, rattus
QQYNNYPLT

SEQ ID NO: 172 - protein, 10 aa, artificial sequence
  Synthetic
GTGGGSGSSS

SEQ ID NO: 173 - protein, 6 aa, artificial sequence
  Synthetic
AAGGSG

SEQ ID NO: 174 - DNA, 1533 bp, artificial sequence
  Synthetic
atgatgtcctttgtctctctgctcctggttggcatcctattccatgccacccaggccctcgaggtgacatgtgaacccggtacgacgtttaaggataagtgcaacacatgtaggtgcggtagcgacggcaaatcagcgttctgtacccggaaattgtgctaccagggaactggaggagggtcggggtcctcgtcacaggtcaccttgaaggagtctggtcctgtgctggtgaaacccacagagaccctcacgctgacctgcaccgtctctgggttctcactcagcaggggtaaaatgggtgtgagctggatccgtcagcccccagggaaggccctggagtggcttgcacacattttttcgagtgacgaaaaatcctacaggacatcgctgaagagcaggctcaccatctccaaggacacctccaaaaaccaggtggtccttacaatgaccaacatggaccctgtggacacagccacgtattactgtgcacggatacgacgtggaggaattgactactggggccagggaaccctggtcactgtctcctcagcctccaccaagggcccatccgtcttccccctggcgccctgctccaggagcacctccgagagcacagccgccctgggctgcctggtcaaggactacttccccgaaccggtgacggtgtcgtggaactcaggcgccctgaccagcggcgtgcacaccttcccggctgtcctacagtcctcaggactctactccctcagcagcgtggtgaccgtgccctccagcagcttgggcacgaagacctacacctgcaacgtagatcacaagcccagcaacaccaaggtggacaagagagttgagtccaaatatggtcccccatgcccaccatgcccagcacctgagttcctggggggaccatcagtcttcctgttccccccaaaacccaaggacactctcatgatctcccggacccctgaggtcacgtgcgtggtggtggacgtgagccaggaagaccccgaggtccagttcaactggtacgtggatggcgtggaggtgcataatgccaagacaaagccgcgggaggagcagttcaacagcacgtaccgtgtggtcagcgtcctcaccgtcctgcaccaggactggctgaacggcaaggagtacaagtgcaaggtctccaacaaaggcctcccgtcctccatcgagaaaaccatctccaaagccaaagggcagccccgagagccacaggtgtacaccctgcccccatcccaggaggagatgaccaagaaccaggtcagcctgacctgcctggtcaaaggcttctaccccagcgacatcgccgtggagtgggagagcaatgggcagccggagaacaactacaagaccacgcctcccgtgctggactccgacggctccttcttcctctacagcaggctaaccgtggacaagagcaggtggcaggaggggaatgtcttctcatgctccgtgatgcatgaggctctgcacaaccactacacacagaagagcctctccctgtctctcgggaaatga

SEQ ID NO: 175 - protein, 491 aa, artificial sequence
  Synthetic
LEVTCEPGTTFKDKCNTCRCGSDGKSAFCTRKLCYQGTGGGSGSSSQVTLKESGPVLVKPTETLTLTCTVSGFSLSRGKMGVSWIRQPPGKALEWLAHIFSSDEKSYRTSLKSRLTISKDTSKNQVVLTMTNMDPVDTATYYCARIRRGGIDYWGQGTLVTVSSASTKGPSVFPLAPCSRSTSESTAALGCLVKDYFPEPVTVSWNSGALTSGVHTFPAVLQSSGLYSLSSVVTVPSSSLGTKTYTCNVDHKPSNTKVDKRVESKYGPPCPPCPAPEFLGGPSVFLFPPKPKDTLMISRTPEVTCVVVDVSQEDPEVQFNWYVDGVEVHNAKTKPREEQFNSTYRVVSVLTVLHQDWLNGKEYKCKVSNKGLPSSIEKTISKAKGQPREPQVYTLPPSQEEMTKNQVSLTCLVKGFYPSDIAVEWESNGQPENNYKTTPPVLDSDGSFFLYSRLTVDKSRWQEGNVFSCSVMHEALHNHYTQKSLSLSLGK

SEQ ID NO: 176 - DNA, 1533 bp, artificial sequence
  Synthetic
atgatgtcctttgtctctctgctcctggttggcatcctattccatgccacccaggccttggaagtgacgtgtgagcccggaacgacattcaaagacaagtgcaatacttgtcggtgcggttcagatgggaaatcggcggtctgcacaaagctctggtgtaaccagggcaccggtggagggtcgggatccagctcacaggtcaccttgaaggagtctggtcctgtgctggtgaaacccacagagaccctcacgctgacctgcaccgtctctgggttctcactcagcaggggtaaaatgggtgtgagctggatccgtcagcccccagggaaggccctggagtggcttgcacacattttttcgagtgacgaaaaatcctacaggacatcgctgaagagcaggctcaccatctccaaggacacctccaaaaaccaggtggtccttacaatgaccaacatggaccctgtggacacagccacgtattactgtgcacggatacgacgtggaggaattgactactggggccagggaaccctggtcactgtctcctcagcctccaccaagggcccatccgtcttccccctggcgccctgctccaggagcacctccgagagcacagccgccctgggctgcctggtcaaggactacttccccgaaccggtgacggtgtcgtggaactcaggcgccctgaccagcggcgtgcacaccttcccggctgtcctacagtcctcaggactctactccctcagcagcgtggtgaccgtgccctccagcagcttgggcacgaagacctacacctgcaacgtagatcacaagcccagcaacaccaaggtggacaagagagttgagtccaaatatggtcccccatgcccaccatgcccagcacctgagttcctggggggaccatcagtcttcctgttccccccaaaacccaaggacactctcatgatctcccggacccctgaggtcacgtgcgtggtggtggacgtgagccaggaagaccccgaggtccagttcaactggtacgtggatggcgtggaggtgcataatgccaagacaaagccgcgggaggagcagttcaacagcacgtaccgtgtggtcagcgtcctcaccgtcctgcaccaggactggctgaacggcaaggagtacaagtgcaaggtctccaacaaaggcctcccgtcctccatcgagaaaaccatctccaaagccaaagggcagccccgagagccacaggtgtacaccctgcccccatcccaggaggagatgaccaagaaccaggtcagcctgacctgcctggtcaaaggcttctaccccagcgacatcgccgtggagtgggagagcaatgggcagccggagaacaactacaagaccacgcctcccgtgctggactccgacggctccttcttcctctacagcaggctaaccgtggacaagagcaggtggcaggaggggaatgtcttctcatgctccgtgatgcatgaggctctgcacaaccactacacacagaagagcctctccctgtctctcgggaaatga

SEQ ID NO: 177 - protein, 491 aa, artificial sequence
  Synthetic
LEVTCEPGTTFKDKCNTCRCGSDGKSAVCTKLWCNQGTGGGSGSSSQVTLKESGPVLVKPTETLTLTCTVSGFSLSRGKMGVSWIRQPPGKALEWLAHIFSSDEKSYRTSLKSRLTISKDTSKNQVVLTMTNMDPVDTATYYCARIRRGGIDYWGQGTLVTVSSASTKGPSVFPLAPCSRSTSESTAALGCLVKDYFPEPVTVSWNSGALTSGVHTFPAVLQSSGLYSLSSVVTVPSSSLGTKTYTCNVDHKPSNTKVDKRVESKYGPPCPPCPAPEFLGGPSVFLFPPKPKDTLMISRTPEVTCVVVDVSQEDPEVQFNWYVDGVEVHNAKTKPREEQFNSTYRVVSVLTVLHQDWLNGKEYKCKVSNKGLPSSIEKTISKAKGQPREPQVYTLPPSQEEMTKNQVSLTCLVKGFYPSDIAVEWESNGQPENNYKTTPPVLDSDGSFFLYSRLTVDKSRWQEGNVFSCSVMHEALHNHYTQKSLSLSLGK

SEQ ID NO: 178 - DNA, 1533 bp, artificial sequence
  Synthetic
atgatgtcctttgtctctctgctcctggttggcatcctattccatgccacccaggcccaggtcaccttgaaggagtctggtcctgtgctggtgaaacccacagagaccctcacgctgacctgcaccgtctctgggttctcactcagcaggggtaaaatgggtgtgagctggatccgtcagcccccagggaaggccctggagtggcttgcacacattttttcgagtgacgaaaaatcctacaggacatcgctgaagagcaggctcaccatctccaaggacacctccaaaaaccaggtggtccttacaatgaccaacatggaccctgtggacacagccacgtattactgtgcacggatacgacgtggaggaattgactactggggccagggaaccctggtcactgtctcctcagcctccaccaagggcccatccgtcttccccctggcgccctgctccaggagcacctccgagagcacagccgccctgggctgcctggtcaaggactacttccccgaaccggtgacggtgtcgtggaactcaggcgccctgaccagcggcgtgcacaccttcccggctgtcctacagtcctcaggactctactccctcagcagcgtggtgaccgtgccctccagcagcttgggcacgaagacctacacctgcaacgtagatcacaagcccagcaacaccaaggtggacaagagagttgagtccaaatatggtcccccatgcccaccatgcccagcacctgagttcctggggggaccatcagtcttcctgttccccccaaaacccaaggacactctcatgatctcccggacccctgaggtcacgtgcgtggtggtggacgtgagccaggaagaccccgaggtccagttcaactggtacgtggatggcgtggaggtgcataatgccaagacaaagccgcgggaggagcagttcaacagcacgtaccgtgtggtcagcgtcctcaccgtcctgcaccaggactggctgaacggcaaggagtacaagtgcaaggtctccaacaaaggcctcccgtcctccatcgagaaaaccatctccaaagccaaagggcagccccgagagccacaggtgtacaccctgcccccatcccaggaggagatgaccaagaaccaggtcagcctgacctgcctggtcaaaggcttctaccccagcgacatcgccgtggagtgggagagcaatgggcagccggagaacaactacaagaccacgcctcccgtgctggactccgacggctccttcttcctctacagcaggctaaccgtggacaagagcaggtggcaggaggggaatgtcttctcatgctccgtgatgcatgaggctctgcacaaccactacacacagaagagcctctccctgtctctcgggaaagccgctggtggtagtggtctcgaggtgacatgtgaacccggtacgacgtttaaggataagtgcaacacatgtaggtgcggtagcgacggcaaatcagcgttctgtacccggaaattgtgctaccagggtagtggtgcttga

SEQ ID NO: 179 - protein, 491 aa, artificial sequence
  Synthetic
QVTLKESGPVLVKPTETLTLTCTVSGFSLSRGKMGVSWIRQPPGKALEWLAHIFSSDEKSYRTSLKSRLTISKDTSKNQVVLTMTNMDPVDTATYYCARIRRGGIDYWGQGTLVTVSSASTKGPSVFPLAPCSRSTSESTAALGCLVKDYFPEPVTVSWNSGALTSGVHTFPAVLQSSGLYSLSSVVTVPSSSLGTKTYTCNVDHKPSNTKVDKRVESKYGPPCPPCPAPEFLGGPSVFLFPPKPKDTLMISRTPEVTCVVVDVSQEDPEVQFNWYVDGVEVHNAKTKPREEQFNSTYRVVSVLTVLHQDWLNGKEYKCKVSNKGLPSSIEKTISKAKGQPREPQVYTLPPSQEEMTKNQVSLTCLVKGFYPSDIAVEWESNGQPENNYKTTPPVLDSDGSFFLYSRLTVDKSRWQEGNVFSCSVMHEALHNHYTQKSLSLSLGKAAGGSGLEVTCEPGTTFKDKCNTCRCGSDGKSAFCTRKLCYQGSGA

SEQ ID NO: 180 - DNA, 1533 bp, artificial sequence
  Synthetic
atgatgtcctttgtctctctgctcctggttggcatcctattccatgccacccaggcccaggtcaccttgaaggagtctggtcctgtgctggtgaaacccacagagaccctcacgctgacctgcaccgtctctgggttctcactcagcaggggtaaaatgggtgtgagctggatccgtcagcccccagggaaggccctggagtggcttgcacacattttttcgagtgacgaaaaatcctacaggacatcgctgaagagcaggctcaccatctccaaggacacctccaaaaaccaggtggtccttacaatgaccaacatggaccctgtggacacagccacgtattactgtgcacggatacgacgtggaggaattgactactggggccagggaaccctggtcactgtctcctcagcctccaccaagggcccatccgtcttccccctggcgccctgctccaggagcacctccgagagcacagccgccctgggctgcctggtcaaggactacttccccgaaccggtgacggtgtcgtggaactcaggcgccctgaccagcggcgtgcacaccttcccggctgtcctacagtcctcaggactctactccctcagcagcgtggtgaccgtgccctccagcagcttgggcacgaagacctacacctgcaacgtagatcacaagcccagcaacaccaaggtggacaagagagttgagtccaaatatggtcccccatgcccaccatgcccagcacctgagttcctggggggaccatcagtcttcctgttccccccaaaacccaaggacactctcatgatctcccggacccctgaggtcacgtgcgtggtggtggacgtgagccaggaagaccccgaggtccagttcaactggtacgtggatggcgtggaggtgcataatgccaagacaaagccgcgggaggagcagttcaacagcacgtaccgtgtggtcagcgtcctcaccgtcctgcaccaggactggctgaacggcaaggagtacaagtgcaaggtctccaacaaaggcctcccgtcctccatcgagaaaaccatctccaaagccaaagggcagccccgagagccacaggtgtacaccctgcccccatcccaggaggagatgaccaagaaccaggtcagcctgacctgcctggtcaaaggcttctaccccagcgacatcgccgtggagtgggagagcaatgggcagccggagaacaactacaagaccacgcctcccgtgctggactccgacggctccttcttcctctacagcaggctaaccgtggacaagagcaggtggcaggaggggaatgtcttctcatgctccgtgatgcatgaggctctgcacaaccactacacacagaagagcctctccctgtctctcgggaaagccgctggtggtagtggtttggaagtgacgtgtgagcccggaacgacattcaaagacaagtgcaatacttgtcggtgcggttcagatgggaaatcggcggtctgcacaaagctctggtgtaaccagggtagtggtgcttga

SEQ ID NO: 181 - protein, 491 aa, artificial sequence
  Synthetic
QVTLKESGPVLVKPTETLTLTCTVSGFSLSRGKMGVSWIRQPPGKALEWLAHIFSSDEKSYRTSLKSRLTISKDTSKNQVVLTMTNMDPVDTATYYCARIRRGGIDYWGQGTLVTVSSASTKGPSVFPLAPCSRSTSESTAALGCLVKDYFPEPVTVSWNSGALTSGVHTFPAVLQSSGLYSLSSVVTVPSSSLGTKTYTCNVDHKPSNTKVDKRVESKYGPPCPPCPAPEFLGGPSVFLFPPKPKDTLMISRTPEVTCVVVDVSQEDPEVQFNWYVDGVEVHNAKTKPREEQFNSTYRVVSVLTVLHQDWLNGKEYKCKVSNKGLPSSIEKTISKAKGQPREPQVYTLPPSQEEMTKNQVSLTCLVKGFYPSDIAVEWESNGQPENNYKTTPPVLDSDGSFFLYSRLTVDKSRWQEGNVFSCSVMHEALHNHYTQKSLSLSLGKAAGGSGLEVTCEPGTTFKDKCNTCRCGSDGKSAVCTKLWCNQGSGA

SEQ ID NO: 182 - DNA, 834 bp, artificial sequence
  Synthetic
atgatgtcctttgtctctctgctcctggttggcatcctattccatgccacccaggccctcgaggtgacatgtgaacccggtacgacgtttaaggataagtgcaacacatgtaggtgcggtagcgacggcaaatcagcgttctgtacccggaaattgtgctaccagggaactggaggagggtcggggtcctcgtcacagccagtgctgactcagcccccctcactgtccgtgtccccaggacagacagccagcatcacctgctctggagagaaattgggggataaatatgcttactggtatcagcagaagccaggccagtcccctgtgttggtcatgtatcaagataaacagcggccctcagggatccctgagcgattctctggctccaactctgggaacacagccactctgaccatcagcgggacccaggctatggatgaggctgactattactgtcaggcgtgggacagcagcactgcggtattcggcggagggaccaagctgaccgtcctaggccagcctaaggcggcgccctcggtcaccctgttcccgccctcctctgaggagcttcaagccaacaaggccacactggtgtgtctcataagtgacttctacccgggagccgtgacagtggcctggaaggcagatagcagccccgtcaaggcgggagtggagaccaccacaccctccaaacaaagcaacaacaagtacgcggccagcagctatctgagcctgacgcctgagcagtggaagtcccacagaagctacagctgccaggtcacgcatgaagggagcaccgtggagaagacagtggcccctacagaatgttcatag

SEQ ID NO: 183 - protein, 258 aa, artificial sequence
  Synthetic
LEVTCEPGTTFKDKCNTCRCGSDGKSAFCTRKLCYQGTGGGSGSSSQPVLTQPPSLSVSPGQTASITCSGEKLGDKYAYWYQQKPGQSPVLVMYQDKQRPSGIPERFSGSNSGNTATLTISGTQAMDEADYYCQAWDSSTAVFGGGTKLTVLGQPKAAPSVTLFPPSSEELQANKATLVCLISDFYPGAVTVAWKADSSPVKAGVETTTPSKQSNNKYAASSYLSLTPEQWKSHRSYSCQVTHEGSTVEKTVAPTECS

SEQ ID NO: 184 - DNA, 834 bp, artificial sequence
  Synthetic
atgatgtcctttgtctctctgctcctggttggcatcctattccatgccacccaggccttggaagtgacgtgtgagcccggaacgacattcaaagacaagtgcaatacttgtcggtgcggttcagatgggaaatcggcggtctgcacaaagctctggtgtaaccagggcaccggtggagggtcgggatccagctcacagccagtgctgactcagcccccctcactgtccgtgtccccaggacagacagccagcatcacctgctctggagagaaattgggggataaatatgcttactggtatcagcagaagccaggccagtcccctgtgttggtcatgtatcaagataaacagcggccctcagggatccctgagcgattctctggctccaactctgggaacacagccactctgaccatcagcgggacccaggctatggatgaggctgactattactgtcaggcgtgggacagcagcactgcggtattcggcggagggaccaagctgaccgtcctaggccagcctaaggcggcgccctcggtcaccctgttcccgccctcctctgaggagcttcaagccaacaaggccacactggtgtgtctcataagtgacttctacccgggagccgtgacagtggcctggaaggcagatagcagccccgtcaaggcgggagtggagaccaccacaccctccaaacaaagcaacaacaagtacgcggccagcagctatctgagcctgacgcctgagcagtggaagtcccacagaagctacagctgccaggtcacgcatgaagggagcaccgtggagaagacagtggcccctacagaatgttcatag

SEQ ID NO: 185 - protein, 258 aa, artificial sequence
  Synthetic
LEVTCEPGTTFKDKCNTCRCGSDGKSAVCTKLWCNQGTGGGSGSSSQPVLTQPPSLSVSPGQTASITCSGEKLGDKYAYWYQQKPGQSPVLVMYQDKQRPSGIPERFSGSNSGNTATLTISGTQAMDEADYYCQAWDSSTAVFGGGTKLTVLGQPKAAPSVTLFPPSSEELQANKATLVCLISDFYPGAVTVAWKADSSPVKAGVETTTPSKQSNNKYAASSYLSLTPEQWKSHRSYSCQVTHEGSTVEKTVAPTECS

SEQ ID NO: 186 - DNA, 834 bp, artificial sequence
  Synthetic
atgatgtcctttgtctctctgctcctggttggcatcctattccatgccacccaggcccagccagtgctgactcagcccccctcactgtccgtgtccccaggacagacagccagcatcacctgctctggagagaaattgggggataaatatgcttactggtatcagcagaagccaggccagtcccctgtgttggtcatgtatcaagataaacagcggccctcagggatccctgagcgattctctggctccaactctgggaacacagccactctgaccatcagcgggacccaggctatggatgaggctgactattactgtcaggcgtgggacagcagcactgcggtattcggcggagggaccaagctgaccgtcctaggccagcctaaggcggcgccctcggtcaccctgttcccgccctcctctgaggagcttcaagccaacaaggccacactggtgtgtctcataagtgacttctacccgggagccgtgacagtggcctggaaggcagatagcagccccgtcaaggcgggagtggagaccaccacaccctccaaacaaagcaacaacaagtacgcggccagcagctatctgagcctgacgcctgagcagtggaagtcccacagaagctacagctgccaggtcacgcatgaagggagcaccgtggagaagacagtggcccctacagaatgttcagccgctggtggtagtggtctcgaggtgacatgtgaacccggtacgacgtttaaggataagtgcaacacatgtaggtgcggtagcgacggcaaatcagcgttctgtacccggaaattgtgctaccagggtagtggtgcttag

SEQ ID NO: 187 - protein, 258 aa, artificial sequence
  Synthetic
QPVLTQPPSLSVSPGQTASITCSGEKLGDKYAYWYQQKPGQSPVLVMYQDKQRPSGIPERFSGSNSGNTATLTISGTQAMDEADYYCQAWDSSTAVFGGGTKLTVLGQPKAAPSVTLFPPSSEELQANKATLVCLISDFYPGAVTVAWKADSSPVKAGVETTTPSKQSNNKYAASSYLSLTPEQWKSHRSYSCQVTHEGSTVEKTVAPTECSAAGGSGLEVTCEPGTTFKDKCNTCRCGSDGKSAFCTRKLCYQGSGA

SEQ ID NO: 188 - DNA, 834 bp, artificial sequence
  Synthetic
atgatgtcctttgtctctctgctcctggttggcatcctattccatgccacccaggcccagccagtgctgactcagcccccctcactgtccgtgtccccaggacagacagccagcatcacctgctctggagagaaattgggggataaatatgcttactggtatcagcagaagccaggccagtcccctgtgttggtcatgtatcaagataaacagcggccctcagggatccctgagcgattctctggctccaactctgggaacacagccactctgaccatcagcgggacccaggctatggatgaggctgactattactgtcaggcgtgggacagcagcactgcggtattcggcggagggaccaagctgaccgtcctaggccagcctaaggcggcgccctcggtcaccctgttcccgccctcctctgaggagcttcaagccaacaaggccacactggtgtgtctcataagtgacttctacccgggagccgtgacagtggcctggaaggcagatagcagccccgtcaaggcgggagtggagaccaccacaccctccaaacaaagcaacaacaagtacgcggccagcagctatctgagcctgacgcctgagcagtggaagtcccacagaagctacagctgccaggtcacgcatgaagggagcaccgtggagaagacagtggcccctacagaatgttcagccgctggtggtagtggtttggaagtgacgtgtgagcccggaacgacattcaaagacaagtgcaatacttgtcggtgcggttcagatgggaaatcggcggtctgcacaaagctctggtgtaaccagggtagtggtgcttag

SEQ ID NO: 189 - protein, 258 aa, artificial sequence
  Synthetic
QPVLTQPPSLSVSPGQTASITCSGEKLGDKYAYWYQQKPGQSPVLVMYQDKQRPSGIPERFSGSNSGNTATLTISGTQAMDEADYYCQAWDSSTAVFGGGTKLTVLGQPKAAPSVTLFPPSSEELQANKATLVCLISDFYPGAVTVAWKADSSPVKAGVETTTPSKQSNNKYAASSYLSLTPEQWKSHRSYSCQVTHEGSTVEKTVAPTECSAAGGSGLEVTCEPGTTFKDKCNTCRCGSDGKSAVCTKLWCNQGSGA

SEQ ID NO: 190 - protein, 501 aa, artificial sequence; identical to SEQ ID NO: 89
  Synthetic

SEQ ID NO: 191 - DNA, 837 bp, artificial sequence; identical to SEQ ID NO: 100
  Synthetic

SEQ ID NO: 192 - protein, 8 aa, Artificial Sequence
  Synthetic
SGGGGSGS

SEQ ID NO: 193 - protein, 9 aa, Artificial Sequence
  Synthetic
SGGGSGGGS

SEQ ID NO: 194 - protein, 12 aa, Artificial Sequence
  Synthetic
GTGGGSGSSSYG

SEQ ID NO: 195 - protein, 6 aa, Artificial Sequence
  Synthetic
GSGSYG